European Patent Application EP 4 198 129 A1, published June 21, 2023. Title: Mutant human alpha-N-acetyl glucosaminidase and use thereof. Applicant: JCR Pharmaceuticals Co., Ltd. The sequence listing filed with the application follows.

SEQUENCE LISTING (67 sequences)

SEQ ID NO: 1 - protein, 720 aa, Homo sapiens
DEAREAAAVRALVARLLGPGPAADFSVSVERALAAKPGLDTYSLGGGGAARVRVRGSTGVAAAAGLHRYLRDFCGCHVAWSGSQLRLPRPLPAVPGELTEATPNRYRYYQNVCTQSYSFVWWDWARWEREIDWMALNGINLALAWSGQEAIWQRVYLALGLTQAEINEFFTGPAFLAWGRMGNLHTWDGPLPPSWHIKQLYLQHRVLDQMRSFGMTPVLPAFAGHVPEAVTRVFPQVNVTKMGSWGHFNCSYSCSFLLAPEDPIFPIIGSLFLRELIKEFGTDHIYGADTFNEMQPPSSEPSYLAAATTAVYEAMTAVDTEAVWLLQGWLFQHQPQFWGPAQIRAVLGAVPRGRLLVLDLFAESQPVYTRTASFQGQPFIWCMLHNFGGNHGLFGALEAVNGGPEAARLFPNSTMVGTGMAPEGISQNEVVYSLMAELGWRKDPVPDLAAWVTSFAARRYGVSHPDAGAAWRLLLRSVYNCSGEACRGHNRSPLVRRPSLQMNTSIWYNRSDVFEAWRLLLTSAPSLATSPAFRYDLLDLTRQAVQELVSLYYEEARSAYLSKELASLLRAGGVLAYELLPALDEVLASDSRFLLGSWLEQARAAAVSEAEADFYEQNSRYQLTLWGPEGNILDYANKQLAGLVANYYTPRWRLFLEALVDSVAQGIPFQQHQFDKNVFQLEQAFVLSKQRYPSQPRGDTVDLAKKIFLKYYPRWVAGSW

SEQ ID NO: 2 - DNA, 2229 bp, Homo sapiens
atggaggctgtggccgtcgccgccgctgtgggcgtgctgctgctggctggcgctggcggcgccgccggcgacgaggctagggaagccgccgccgtgcgggccctcgtggctaggctgctgggccccggtcccgctgccgatttttccgtgagcgtcgagagggccctcgctgctaagcccggtttagacacctactccctcggcggaggaggagctgctagggttcgtgttcgtggatccactggtgtggccgctgctgctggactccatcgttatttacgggatttctgtggatgccacgtggcttggagcggcagccaactgaggctccctaggcctctgcccgctgtccccggtgaactgaccgaggctacccccaatcggtaccggtactaccagaacgtgtgcacccaaagctattccttcgtgtggtgggactgggctcgttgggaaagggagatcgactggatggccctcaacggaattaatctggctttagcttggtccggccaagaggccatttggcagagggtgtacctcgctttaggtttaacacaagctgagatcaacgaattcttcaccggccccgcttttctcgcttggggacggatgggcaatttacacacttgggatggccctctccccccttcttggcacattaagcaactgtatttacagcatcgtgtgctcgatcagatgaggtccttcggcatgacacccgtgctccccgcttttgctggccacgtccccgaagctgtcactcgtgtgtttcctcaagttaacgtgacaaagatgggctcttggggccactttaactgcagctacagctgttcctttttactggcccccgaggatcccatttttcccatcatcggctccctctttttaagggagctgatcaaagagttcggcaccgaccacatttacggcgccgacacctttaacgagatgcagccccctagcagcgagcctagctatttagctgctgccaccacagccgtctatgaggccatgaccgccgtggacaccgaagctgtgtggctgctgcaaggttggctgttccagcaccagcctcagttctggggccccgctcaaattcgtgccgtgctgggcgccgtgcctcggggtcgtctgctggtcctcgatctgttcgctgagtcccaacccgtttacacaaggacagcctccttccaaggtcagcccttcatctggtgcatgctgcacaactttggcggaaaccacggactgttcggagctttagaggctgtgaatggcggacccgaagctgcccggctgttccccaactccaccatggtgggaaccggaatggcccccgaaggcatttcccagaatgaggtggtctacagcctcatggccgagctcggatggcggaaggatcccgttcccgatttagctgcttgggtgacctccttcgctgctcggaggtatggcgtgtcccatcccgatgccggagctgcttggaggttattattacgttccgtctacaactgctccggcgaggcttgccggggacataatcggtcccctttagttcgtaggccttctttacagatgaataccagcatctggtacaaccggagcgacgtgttcgaagcttggcgtttattactgacatccgctccctctttagctaccagccccgcctttcgttatgatttattagatctgactcgtcaagctgtgcaagaactggtgtctttatactacgaggaagctcggagcgcctatttatccaaagagctggcctctttactgagggctggaggcgtgctggcttatgagctgctccccgctttagatgaggttttagctagcgactctcgttttttactgggatcttggctggagcaagctcgtgccgctgccgtgagcgaagccgaggccgatttctatgagcagaactcccggtaccagctgacactctggggccccgagggcaacattctggactacgccaacaagcagctggctggactggtggccaactactacacccctcgttggaggctgtttttagaagctctggtcgactccgtggcccaaggtatccccttccaacagcaccagttcgacaagaatgtgttccagctggaacaagctttcgtgctgtccaaacaaaggtacccctcccagccccggggagacacagtggatctggccaagaagatctttttaaagtattaccctcggtgggtggctggaagctgg

SEQ ID NO: 3 - protein, 720 aa, Artificial Sequence
  amino acid sequence of  hNAGLU mutant type 1
DEAREAAAVRALVARLLGPGPAADFSVSVERALAAESGLDTYSLGGGGAARVRVRGSTGVAAAAGLHRYLRDFCGCHVAWSGSQLRLPRPLPAVPGELTEATPNRYRYYQNVCTQSYSFVWWDWARWEREIDWMALNGINLALAWSGQEAIWQRVYLALGLTQAEINEFFTGPAFLAWGRMGNLHTWDGPLPPSWHIKQLYLQHRVLDQMRSFGMTPVLPAFAGHVPEAVTRVFPQVNVTKMGSWGHFNCSYSCSFLLAPEDPIFPIIGSLFLRELIKEFGTDHIYGADTFNEMQPPSSEPSYLAAATTAVYEAMTAVDTEAVWLLQGWLFQHQPQFWGPAQIRAVLGAVPRGRLLVLDLFAESQPVYTRTASFQGQPFIWCMLHNFGGNHGLFGALEAVNGGPEAARLFPNSTMVGTGMAPEGISQNEVVYSLMAELGWRKDPVPDLAAWVTSFAARRYGVSHPDAGAAWRLLLRSVYNCSGEACRGHNRSPLVRRPSLQMNTSIWYNRSDVFEAWRLLLTSAPSLATSPAFRYDLLDLTRQAVQELVSLYYEEARSAYLSKELASLLRAGGVLAYELLPALDEVLASDSRFLLGSWLEQARAAAVSEAEADFYEQNSRYQLTLWGPEGNILDYANKQLAGLVANYYTPRWRLFLEALVDSVAQGIPFQQHQFDKNVFQLEQAFVLSKQRYPSQPRGDTVDLAKKIFLKYYPRWVAGSW

SEQ ID NO: 4 - DNA, 2229 bp, Artificial Sequence
  nucleic acid sequence coding hNAGLU mutant type 1, synthetic sequence
atggaggctgtggccgtcgccgccgctgtgggcgtgctgctgctggctggcgctggcggcgccgccggcgacgaggctagggaagccgccgccgtgcgggccctcgtggctaggctgctgggccccggtcccgctgccgatttttccgtgagcgtcgagagggccctcgctgctgagtccggtttagacacctactccctcggcggaggaggagctgctagggttcgtgttcgtggatccactggtgtggccgctgctgctggactccatcgttatttacgggatttctgtggatgccacgtggcttggagcggcagccaactgaggctccctaggcctctgcccgctgtccccggtgaactgaccgaggctacccccaatcggtaccggtactaccagaacgtgtgcacccaaagctattccttcgtgtggtgggactgggctcgttgggaaagggagatcgactggatggccctcaacggaattaatctggctttagcttggtccggccaagaggccatttggcagagggtgtacctcgctttaggtttaacacaagctgagatcaacgaattcttcaccggccccgcttttctcgcttggggacggatgggcaatttacacacttgggatggccctctccccccttcttggcacattaagcaactgtatttacagcatcgtgtgctcgatcagatgaggtccttcggcatgacacccgtgctccccgcttttgctggccacgtccccgaagctgtcactcgtgtgtttcctcaagttaacgtgacaaagatgggctcttggggccactttaactgcagctacagctgttcctttttactggcccccgaggatcccatttttcccatcatcggctccctctttttaagggagctgatcaaagagttcggcaccgaccacatttacggcgccgacacctttaacgagatgcagccccctagcagcgagcctagctatttagctgctgccaccacagccgtctatgaggccatgaccgccgtggacaccgaagctgtgtggctgctgcaaggttggctgttccagcaccagcctcagttctggggccccgctcaaattcgtgccgtgctgggcgccgtgcctcggggtcgtctgctggtcctcgatctgttcgctgagtcccaacccgtttacacaaggacagcctccttccaaggtcagcccttcatctggtgcatgctgcacaactttggcggaaaccacggactgttcggagctttagaggctgtgaatggcggacccgaagctgcccggctgttccccaactccaccatggtgggaaccggaatggcccccgaaggcatttcccagaatgaggtggtctacagcctcatggccgagctcggatggcggaaggatcccgttcccgatttagctgcttgggtgacctccttcgctgctcggaggtatggcgtgtcccatcccgatgccggagctgcttggaggttattattacgttccgtctacaactgctccggcgaggcttgccggggacataatcggtcccctttagttcgtaggccttctttacagatgaataccagcatctggtacaaccggagcgacgtgttcgaagcttggcgtttattactgacatccgctccctctttagctaccagccccgcctttcgttatgatttattagatctgactcgtcaagctgtgcaagaactggtgtctttatactacgaggaagctcggagcgcctatttatccaaagagctggcctctttactgagggctggaggcgtgctggcttatgagctgctccccgctttagatgaggttttagctagcgactctcgttttttactgggatcttggctggagcaagctcgtgccgctgccgtgagcgaagccgaggccgatttctatgagcagaactcccggtaccagctgacactctggggccccgagggcaacattctggactacgccaacaagcagctggctggactggtggccaactactacacccctcgttggaggctgtttttagaagctctggtcgactccgtggcccaaggtatccccttccaacagcaccagttcgacaagaatgtgttccagctggaacaagctttcgtgctgtccaaacaaaggtacccctcccagccccggggagacacagtggatctggccaagaagatctttttaaagtattaccctcggtgggtggctggaagctgg

SEQ ID NO: 5 - protein, 721 aa, Artificial Sequence
  amino acid sequence of  hNAGLU mutant type 2
DEAREAAAVRALVARLLGPGPAADFSVSVERALAAKPGLDTYSLSGGGGAARVRVRGSTGVAAAAGLHRYLRDFCGCHVAWSGSQLRLPRPLPAVPGELTEATPNRYRYYQNVCTQSYSFVWWDWARWEREIDWMALNGINLALAWSGQEAIWQRVYLALGLTQAEINEFFTGPAFLAWGRMGNLHTWDGPLPPSWHIKQLYLQHRVLDQMRSFGMTPVLPAFAGHVPEAVTRVFPQVNVTKMGSWGHFNCSYSCSFLLAPEDPIFPIIGSLFLRELIKEFGTDHIYGADTFNEMQPPSSEPSYLAAATTAVYEAMTAVDTEAVWLLQGWLFQHQPQFWGPAQIRAVLGAVPRGRLLVLDLFAESQPVYTRTASFQGQPFIWCMLHNFGGNHGLFGALEAVNGGPEAARLFPNSTMVGTGMAPEGISQNEVVYSLMAELGWRKDPVPDLAAWVTSFAARRYGVSHPDAGAAWRLLLRSVYNCSGEACRGHNRSPLVRRPSLQMNTSIWYNRSDVFEAWRLLLTSAPSLATSPAFRYDLLDLTRQAVQELVSLYYEEARSAYLSKELASLLRAGGVLAYELLPALDEVLASDSRFLLGSWLEQARAAAVSEAEADFYEQNSRYQLTLWGPEGNILDYANKQLAGLVANYYTPRWRLFLEALVDSVAQGIPFQQHQFDKNVFQLEQAFVLSKQRYPSQPRGDTVDLAKKIFLKYYPRWVAGSW

SEQ ID NO: 6 - DNA, 2232 bp, Artificial Sequence
  nucleic acid sequence coding hNAGLU mutant type 2, synthetic sequence
atggaggctgtggccgtcgccgccgctgtgggcgtgctgctgctggctggcgctggcggcgccgccggcgacgaggctagggaagccgccgccgtgcgggccctcgtggctaggctgctgggccccggtcccgctgccgatttttccgtgagcgtcgagagggccctcgctgctaagcccggtttagacacctactccctctctggcggaggaggagctgctagggttcgtgttcgtggatccactggtgtggccgctgctgctggactccatcgttatttacgggatttctgtggatgccacgtggcttggagcggcagccaactgaggctccctaggcctctgcccgctgtccccggtgaactgaccgaggctacccccaatcggtaccggtactaccagaacgtgtgcacccaaagctattccttcgtgtggtgggactgggctcgttgggaaagggagatcgactggatggccctcaacggaattaatctggctttagcttggtccggccaagaggccatttggcagagggtgtacctcgctttaggtttaacacaagctgagatcaacgaattcttcaccggccccgcttttctcgcttggggacggatgggcaatttacacacttgggatggccctctccccccttcttggcacattaagcaactgtatttacagcatcgtgtgctcgatcagatgaggtccttcggcatgacacccgtgctccccgcttttgctggccacgtccccgaagctgtcactcgtgtgtttcctcaagttaacgtgacaaagatgggctcttggggccactttaactgcagctacagctgttcctttttactggcccccgaggatcccatttttcccatcatcggctccctctttttaagggagctgatcaaagagttcggcaccgaccacatttacggcgccgacacctttaacgagatgcagccccctagcagcgagcctagctatttagctgctgccaccacagccgtctatgaggccatgaccgccgtggacaccgaagctgtgtggctgctgcaaggttggctgttccagcaccagcctcagttctggggccccgctcaaattcgtgccgtgctgggcgccgtgcctcggggtcgtctgctggtcctcgatctgttcgctgagtcccaacccgtttacacaaggacagcctccttccaaggtcagcccttcatctggtgcatgctgcacaactttggcggaaaccacggactgttcggagctttagaggctgtgaatggcggacccgaagctgcccggctgttccccaactccaccatggtgggaaccggaatggcccccgaaggcatttcccagaatgaggtggtctacagcctcatggccgagctcggatggcggaaggatcccgttcccgatttagctgcttgggtgacctccttcgctgctcggaggtatggcgtgtcccatcccgatgccggagctgcttggaggttattattacgttccgtctacaactgctccggcgaggcttgccggggacataatcggtcccctttagttcgtaggccttctttacagatgaataccagcatctggtacaaccggagcgacgtgttcgaagcttggcgtttattactgacatccgctccctctttagctaccagccccgcctttcgttatgatttattagatctgactcgtcaagctgtgcaagaactggtgtctttatactacgaggaagctcggagcgcctatttatccaaagagctggcctctttactgagggctggaggcgtgctggcttatgagctgctccccgctttagatgaggttttagctagcgactctcgttttttactgggatcttggctggagcaagctcgtgccgctgccgtgagcgaagccgaggccgatttctatgagcagaactcccggtaccagctgacactctggggccccgagggcaacattctggactacgccaacaagcagctggctggactggtggccaactactacacccctcgttggaggctgtttttagaagctctggtcgactccgtggcccaaggtatccccttccaacagcaccagttcgacaagaatgtgttccagctggaacaagctttcgtgctgtccaaacaaaggtacccctcccagccccggggagacacagtggatctggccaagaagatctttttaaagtattaccctcggtgggtggctggaagctgg

SEQ ID NO: 7 - protein, 720 aa, Artificial Sequence
  amino acid sequence of  hNAGLU mutant type 16
DEAREAAAVRALVARLLGPGPAADFSVSVERALAAKPGLDTYSLGGGGAARVRVRGSTGVAAAAGLHRYLRDFCGCHVAWSGSQLRLPRPLPAVPGELTEATPNRYRYYQNVCTQSYSFVWWDWARWEQEIDWMALNGINLALAWSGQEAIWQRVYLALGLTQAEINEFFTGPAFLAWGRMGNLHTWDGPLPPSWHIKQLYLQHRVLDQMRSFGMTPVLPAFAGHVPEAVTRVFPQVNVTKMGSWGHFNCSYSCSFLLAPEDPIFPIIGSLFLRELIKEFGTDHIYGADTFNEMQPPSSEPSYLAAATTAVYEAMTAVDTEAVWLLQGWLFQHQPQFWGPAQIRAVLGAVPRGRLLVLDLFAESQPVYTRTASFQGQPFIWCMLHNFGGNHGLFGALEAVNGGPEAARLFPNSTMVGTGMAPEGISQNEVVYSLMAELGWRKDPVPDLAAWVTSFAARRYGVSHPDAGAAWRLLLRSVYNCSGEACRGHNRSPLVRRPSLQMNTSIWYNRSDVFEAWRLLLTSAPSLATSPAFRYDLLDLTRQAVQELVSLYYEEARSAYLSKELASLLRAGGVLAYELLPALDEVLASDSRFLLGSWLEQARAAAVSEAEADFYEQNSRYQLTLWGPEGNILDYANKQLAGLVANYYTPRWRLFLEALVDSVAQGIPFQQHQFDKNVFQLEQAFVLSKQRYPSQPRGDTVDLAKKIFLKYYPRWVAGSW

SEQ ID NO: 8 - DNA, 2229 bp, Artificial Sequence
  nucleic acid sequence coding hNAGLU mutant type 16, synthetic sequence
atggaggctgtggccgtcgccgccgctgtgggcgtgctgctgctggctggcgctggcggcgccgccggcgacgaggctagggaagccgccgccgtgcgggccctcgtggctaggctgctgggccccggtcccgctgccgatttttccgtgagcgtcgagagggccctcgctgctaagcccggtttagacacctactccctcggcggaggaggagctgctagggttcgtgttcgtggatccactggtgtggccgctgctgctggactccatcgttatttacgggatttctgtggatgccacgtggcttggagcggcagccaactgaggctccctaggcctctgcccgctgtccccggtgaactgaccgaggctacccccaatcggtaccggtactaccagaacgtgtgcacccaaagctattccttcgtgtggtgggactgggctcgttgggaacaggagatcgactggatggccctcaacggaattaatctggctttagcttggtccggccaagaggccatttggcagagggtgtacctcgctttaggtttaacacaagctgagatcaacgaattcttcaccggccccgcttttctcgcttggggacggatgggcaatttacacacttgggatggccctctccccccttcttggcacattaagcaactgtatttacagcatcgtgtgctcgatcagatgaggtccttcggcatgacacccgtgctccccgcttttgctggccacgtccccgaagctgtcactcgtgtgtttcctcaagttaacgtgacaaagatgggctcttggggccactttaactgcagctacagctgttcctttttactggcccccgaggatcccatttttcccatcatcggctccctctttttaagggagctgatcaaagagttcggcaccgaccacatttacggcgccgacacctttaacgagatgcagccccctagcagcgagcctagctatttagctgctgccaccacagccgtctatgaggccatgaccgccgtggacaccgaagctgtgtggctgctgcaaggttggctgttccagcaccagcctcagttctggggccccgctcaaattcgtgccgtgctgggcgccgtgcctcggggtcgtctgctggtcctcgatctgttcgctgagtcccaacccgtttacacaaggacagcctccttccaaggtcagcccttcatctggtgcatgctgcacaactttggcggaaaccacggactgttcggagctttagaggctgtgaatggcggacccgaagctgcccggctgttccccaactccaccatggtgggaaccggaatggcccccgaaggcatttcccagaatgaggtggtctacagcctcatggccgagctcggatggcggaaggatcccgttcccgatttagctgcttgggtgacctccttcgctgctcggaggtatggcgtgtcccatcccgatgccggagctgcttggaggttattattacgttccgtctacaactgctccggcgaggcttgccggggacataatcggtcccctttagttcgtaggccttctttacagatgaataccagcatctggtacaaccggagcgacgtgttcgaagcttggcgtttattactgacatccgctccctctttagctaccagccccgcctttcgttatgatttattagatctgactcgtcaagctgtgcaagaactggtgtctttatactacgaggaagctcggagcgcctatttatccaaagagctggcctctttactgagggctggaggcgtgctggcttatgagctgctccccgctttagatgaggttttagctagcgactctcgttttttactgggatcttggctggagcaagctcgtgccgctgccgtgagcgaagccgaggccgatttctatgagcagaactcccggtaccagctgacactctggggccccgagggcaacattctggactacgccaacaagcagctggctggactggtggccaactactacacccctcgttggaggctgtttttagaagctctggtcgactccgtggcccaaggtatccccttccaacagcaccagttcgacaagaatgtgttccagctggaacaagctttcgtgctgtccaaacaaaggtacccctcccagccccggggagacacagtggatctggccaagaagatctttttaaagtattaccctcggtgggtggctggaagctgg

SEQ ID NO: 9 - protein, 720 aa, Artificial Sequence
  amino acid sequence of  hNAGLU mutant type 3
DEAREAAAVRALVARLLGPGPAADFSVSVERALAAKPGLDTYSLGGGGAARVRVRGSTGVAAAAGLHRYLRDFCGCHVAWSGSQLRLPRPLPAVPGELTEATPNRYRYYQNVCTQSYSFVWWDWARWEREIDWMALNGINLALAWSGQEAIWQRVYLALGLTQAEINEFFTGPAFLAWGRMGNLHTWDGPLPPSWHIKQLYLQHRVLDRMRSFGMTPVLPAFAGHVPEAVTRVFPQVNVTKMGSWGHFNCSYSCSFLLAPEDPIFPIIGSLFLRELIKEFGTDHIYGADTFNEMQPPSSEPSYLAAATTAVYEAMTAVDTEAVWLLQGWLFQHQPQFWGPAQIRAVLGAVPRGRLLVLDLFAESQPVYTRTASFQGQPFIWCMLHNFGGNHGLFGALEAVNGGPEAARLFPNSTMVGTGMAPEGISQNEVVYSLMAELGWRKDPVPDLAAWVTSFAARRYGVSHPDAGAAWRLLLRSVYNCSGEACRGHNRSPLVRRPSLQMNTSIWYNRSDVFEAWRLLLTSAPSLATSPAFRYDLLDLTRQAVQELVSLYYEEARSAYLSKELASLLRAGGVLAYELLPALDEVLASDSRFLLGSWLEQARAAAVSEAEADFYEQNSRYQLTLWGPEGNILDYANKQLAGLVANYYTPRWRLFLEALVDSVAQGIPFQQHQFDKNVFQLEQAFVLSKQRYPSQPRGDTVDLAKKIFLKYYPRWVAGSW

SEQ ID NO: 10 - DNA, 2229 bp, Artificial Sequence
  nucleic acid sequence coding hNAGLU mutant type 3, synthetic sequence
atggaggctgtggccgtcgccgccgctgtgggcgtgctgctgctggctggcgctggcggcgccgccggcgacgaggctagggaagccgccgccgtgcgggccctcgtggctaggctgctgggccccggtcccgctgccgatttttccgtgagcgtcgagagggccctcgctgctaagcccggtttagacacctactccctcggcggaggaggagctgctagggttcgtgttcgtggatccactggtgtggccgctgctgctggactccatcgttatttacgggatttctgtggatgccacgtggcttggagcggcagccaactgaggctccctaggcctctgcccgctgtccccggtgaactgaccgaggctacccccaatcggtaccggtactaccagaacgtgtgcacccaaagctattccttcgtgtggtgggactgggctcgttgggaaagggagatcgactggatggccctcaacggaattaatctggctttagcttggtccggccaagaggccatttggcagagggtgtacctcgctttaggtttaacacaagctgagatcaacgaattcttcaccggccccgcttttctcgcttggggacggatgggcaatttacacacttgggatggccctctccccccttcttggcacattaagcaactgtatttacagcatcgtgtgctcgatcggatgaggtccttcggcatgacacccgtgctccccgcttttgctggccacgtccccgaagctgtcactcgtgtgtttcctcaagttaacgtgacaaagatgggctcttggggccactttaactgcagctacagctgttcctttttactggcccccgaggatcccatttttcccatcatcggctccctctttttaagggagctgatcaaagagttcggcaccgaccacatttacggcgccgacacctttaacgagatgcagccccctagcagcgagcctagctatttagctgctgccaccacagccgtctatgaggccatgaccgccgtggacaccgaagctgtgtggctgctgcaaggttggctgttccagcaccagcctcagttctggggccccgctcaaattcgtgccgtgctgggcgccgtgcctcggggtcgtctgctggtcctcgatctgttcgctgagtcccaacccgtttacacaaggacagcctccttccaaggtcagcccttcatctggtgcatgctgcacaactttggcggaaaccacggactgttcggagctttagaggctgtgaatggcggacccgaagctgcccggctgttccccaactccaccatggtgggaaccggaatggcccccgaaggcatttcccagaatgaggtggtctacagcctcatggccgagctcggatggcggaaggatcccgttcccgatttagctgcttgggtgacctccttcgctgctcggaggtatggcgtgtcccatcccgatgccggagctgcttggaggttattattacgttccgtctacaactgctccggcgaggcttgccggggacataatcggtcccctttagttcgtaggccttctttacagatgaataccagcatctggtacaaccggagcgacgtgttcgaagcttggcgtttattactgacatccgctccctctttagctaccagccccgcctttcgttatgatttattagatctgactcgtcaagctgtgcaagaactggtgtctttatactacgaggaagctcggagcgcctatttatccaaagagctggcctctttactgagggctggaggcgtgctggcttatgagctgctccccgctttagatgaggttttagctagcgactctcgttttttactgggatcttggctggagcaagctcgtgccgctgccgtgagcgaagccgaggccgatttctatgagcagaactcccggtaccagctgacactctggggccccgagggcaacattctggactacgccaacaagcagctggctggactggtggccaactactacacccctcgttggaggctgtttttagaagctctggtcgactccgtggcccaaggtatccccttccaacagcaccagttcgacaagaatgtgttccagctggaacaagctttcgtgctgtccaaacaaaggtacccctcccagccccggggagacacagtggatctggccaagaagatctttttaaagtattaccctcggtgggtggctggaagctgg

SEQ ID NO: 11 - protein, 720 aa, Artificial Sequence
  amino acid sequence of  hNAGLU mutant type 4
DEAREAAAVRALVARLLGPGPAADFSVSVERALAAKPGLDTYSLGGGGAARVRVRGSTGVAAAAGLHRYLRDFCGCHVAWSGSQLRLPRPLPAVPGELTEATPNRYRYYQNVCTQSYSFVWWDWARWEREIDWMALNGINLALAWSGQEAIWQRVYLALGLTQAEINEFFTGPAFLAWGRMGNLHTWDGPLPPSWHIKQLYLQHRVLDQMRSFGMTPVLPAFAGHVPKAVTRVFPQVNVTKMGSWGHFNCSYSCSFLLAPEDPIFPIIGSLFLRELIKEFGTDHIYGADTFNEMQPPSSEPSYLAAATTAVYEAMTAVDTEAVWLLQGWLFQHQPQFWGPAQIRAVLGAVPRGRLLVLDLFAESQPVYTRTASFQGQPFIWCMLHNFGGNHGLFGALEAVNGGPEAARLFPNSTMVGTGMAPEGISQNEVVYSLMAELGWRKDPVPDLAAWVTSFAARRYGVSHPDAGAAWRLLLRSVYNCSGEACRGHNRSPLVRRPSLQMNTSIWYNRSDVFEAWRLLLTSAPSLATSPAFRYDLLDLTRQAVQELVSLYYEEARSAYLSKELASLLRAGGVLAYELLPALDEVLASDSRFLLGSWLEQARAAAVSEAEADFYEQNSRYQLTLWGPEGNILDYANKQLAGLVANYYTPRWRLFLEALVDSVAQGIPFQQHQFDKNVFQLEQAFVLSKQRYPSQPRGDTVDLAKKIFLKYYPRWVAGSW

SEQ ID NO: 12 - DNA, 2229 bp, Artificial Sequence
  nucleic acid sequence coding hNAGLU mutant type 4, synthetic sequence
atggaggctgtggccgtcgccgccgctgtgggcgtgctgctgctggctggcgctggcggcgccgccggcgacgaggctagggaagccgccgccgtgcgggccctcgtggctaggctgctgggccccggtcccgctgccgatttttccgtgagcgtcgagagggccctcgctgctaagcccggtttagacacctactccctcggcggaggaggagctgctagggttcgtgttcgtggatccactggtgtggccgctgctgctggactccatcgttatttacgggatttctgtggatgccacgtggcttggagcggcagccaactgaggctccctaggcctctgcccgctgtccccggtgaactgaccgaggctacccccaatcggtaccggtactaccagaacgtgtgcacccaaagctattccttcgtgtggtgggactgggctcgttgggaaagggagatcgactggatggccctcaacggaattaatctggctttagcttggtccggccaagaggccatttggcagagggtgtacctcgctttaggtttaacacaagctgagatcaacgaattcttcaccggccccgcttttctcgcttggggacggatgggcaatttacacacttgggatggccctctccccccttcttggcacattaagcaactgtatttacagcatcgtgtgctcgatcagatgaggtccttcggcatgacacccgtgctccccgcttttgctggccacgtccccaaagctgtcactcgtgtgtttcctcaagttaacgtgacaaagatgggctcttggggccactttaactgcagctacagctgttcctttttactggcccccgaggatcccatttttcccatcatcggctccctctttttaagggagctgatcaaagagttcggcaccgaccacatttacggcgccgacacctttaacgagatgcagccccctagcagcgagcctagctatttagctgctgccaccacagccgtctatgaggccatgaccgccgtggacaccgaagctgtgtggctgctgcaaggttggctgttccagcaccagcctcagttctggggccccgctcaaattcgtgccgtgctgggcgccgtgcctcggggtcgtctgctggtcctcgatctgttcgctgagtcccaacccgtttacacaaggacagcctccttccaaggtcagcccttcatctggtgcatgctgcacaactttggcggaaaccacggactgttcggagctttagaggctgtgaatggcggacccgaagctgcccggctgttccccaactccaccatggtgggaaccggaatggcccccgaaggcatttcccagaatgaggtggtctacagcctcatggccgagctcggatggcggaaggatcccgttcccgatttagctgcttgggtgacctccttcgctgctcggaggtatggcgtgtcccatcccgatgccggagctgcttggaggttattattacgttccgtctacaactgctccggcgaggcttgccggggacataatcggtcccctttagttcgtaggccttctttacagatgaataccagcatctggtacaaccggagcgacgtgttcgaagcttggcgtttattactgacatccgctccctctttagctaccagccccgcctttcgttatgatttattagatctgactcgtcaagctgtgcaagaactggtgtctttatactacgaggaagctcggagcgcctatttatccaaagagctggcctctttactgagggctggaggcgtgctggcttatgagctgctccccgctttagatgaggttttagctagcgactctcgttttttactgggatcttggctggagcaagctcgtgccgctgccgtgagcgaagccgaggccgatttctatgagcagaactcccggtaccagctgacactctggggccccgagggcaacattctggactacgccaacaagcagctggctggactggtggccaactactacacccctcgttggaggctgtttttagaagctctggtcgactccgtggcccaaggtatccccttccaacagcaccagttcgacaagaatgtgttccagctggaacaagctttcgtgctgtccaaacaaaggtacccctcccagccccggggagacacagtggatctggccaagaagatctttttaaagtattaccctcggtgggtggctggaagctgg

SEQ ID NO: 13 - protein, 720 aa, Artificial Sequence
  amino acid sequence of  hNAGLU mutant type 17
DEAREAAAVRALVARLLGPGPAADFSVSVERALAAKPGLDTYSLGGGGAARVRVRGSTGVAAAAGLHRYLRDFCGCHVAWSGSQLRLPRPLPAVPGELTEATPNRYRYYQNVCTQSYSFVWWDWARWEREIDWMALNGINLALAWSGQEAIWQRVYLALGLTQAEINEFFTGPAFLAWGRMGNLHTWDGPLPPSWHIKQLYLQHRVLDQMRSFGMTPVLPAFAGHVPEAVTRVFPQVNVVKMGSWGHFNCSYSCSFLLAPEDPIFPIIGSLFLRELIKEFGTDHIYGADTFNEMQPPSSEPSYLAAATTAVYEAMTAVDTEAVWLLQGWLFQHQPQFWGPAQIRAVLGAVPRGRLLVLDLFAESQPVYTRTASFQGQPFIWCMLHNFGGNHGLFGALEAVNGGPEAARLFPNSTMVGTGMAPEGISQNEVVYSLMAELGWRKDPVPDLAAWVTSFAARRYGVSHPDAGAAWRLLLRSVYNCSGEACRGHNRSPLVRRPSLQMNTSIWYNRSDVFEAWRLLLTSAPSLATSPAFRYDLLDLTRQAVQELVSLYYEEARSAYLSKELASLLRAGGVLAYELLPALDEVLASDSRFLLGSWLEQARAAAVSEAEADFYEQNSRYQLTLWGPEGNILDYANKQLAGLVANYYTPRWRLFLEALVDSVAQGIPFQQHQFDKNVFQLEQAFVLSKQRYPSQPRGDTVDLAKKIFLKYYPRWVAGSW

SEQ ID NO: 14 - DNA, 2229 bp, Artificial Sequence
  nucleic acid sequence coding hNAGLU mutant type 17, synthetic sequence
atggaggctgtggccgtcgccgccgctgtgggcgtgctgctgctggctggcgctggcggcgccgccggcgacgaggctagggaagccgccgccgtgcgggccctcgtggctaggctgctgggccccggtcccgctgccgatttttccgtgagcgtcgagagggccctcgctgctaagcccggtttagacacctactccctcggcggaggaggagctgctagggttcgtgttcgtggatccactggtgtggccgctgctgctggactccatcgttatttacgggatttctgtggatgccacgtggcttggagcggcagccaactgaggctccctaggcctctgcccgctgtccccggtgaactgaccgaggctacccccaatcggtaccggtactaccagaacgtgtgcacccaaagctattccttcgtgtggtgggactgggctcgttgggaaagggagatcgactggatggccctcaacggaattaatctggctttagcttggtccggccaagaggccatttggcagagggtgtacctcgctttaggtttaacacaagctgagatcaacgaattcttcaccggccccgcttttctcgcttggggacggatgggcaatttacacacttgggatggccctctccccccttcttggcacattaagcaactgtatttacagcatcgtgtgctcgatcagatgaggtccttcggcatgacacccgtgctccccgcttttgctggccacgtccccgaagctgtcactcgtgtgtttcctcaagttaacgtggtcaagatgggctcttggggccactttaactgcagctacagctgttcctttttactggcccccgaggatcccatttttcccatcatcggctccctctttttaagggagctgatcaaagagttcggcaccgaccacatttacggcgccgacacctttaacgagatgcagccccctagcagcgagcctagctatttagctgctgccaccacagccgtctatgaggccatgaccgccgtggacaccgaagctgtgtggctgctgcaaggttggctgttccagcaccagcctcagttctggggccccgctcaaattcgtgccgtgctgggcgccgtgcctcggggtcgtctgctggtcctcgatctgttcgctgagtcccaacccgtttacacaaggacagcctccttccaaggtcagcccttcatctggtgcatgctgcacaactttggcggaaaccacggactgttcggagctttagaggctgtgaatggcggacccgaagctgcccggctgttccccaactccaccatggtgggaaccggaatggcccccgaaggcatttcccagaatgaggtggtctacagcctcatggccgagctcggatggcggaaggatcccgttcccgatttagctgcttgggtgacctccttcgctgctcggaggtatggcgtgtcccatcccgatgccggagctgcttggaggttattattacgttccgtctacaactgctccggcgaggcttgccggggacataatcggtcccctttagttcgtaggccttctttacagatgaataccagcatctggtacaaccggagcgacgtgttcgaagcttggcgtttattactgacatccgctccctctttagctaccagccccgcctttcgttatgatttattagatctgactcgtcaagctgtgcaagaactggtgtctttatactacgaggaagctcggagcgcctatttatccaaagagctggcctctttactgagggctggaggcgtgctggcttatgagctgctccccgctttagatgaggttttagctagcgactctcgttttttactgggatcttggctggagcaagctcgtgccgctgccgtgagcgaagccgaggccgatttctatgagcagaactcccggtaccagctgacactctggggccccgagggcaacattctggactacgccaacaagcagctggctggactggtggccaactactacacccctcgttggaggctgtttttagaagctctggtcgactccgtggcccaaggtatccccttccaacagcaccagttcgacaagaatgtgttccagctggaacaagctttcgtgctgtccaaacaaaggtacccctcccagccccggggagacacagtggatctggccaagaagatctttttaaagtattaccctcggtgggtggctggaagctgg

SEQ ID NO: 15 - protein, 720 aa, Artificial Sequence
  amino acid sequence of  hNAGLU mutant type 5
DEAREAAAVRALVARLLGPGPAADFSVSVERALAAKPGLDTYSLGGGGAARVRVRGSTGVAAAAGLHRYLRDFCGCHVAWSGSQLRLPRPLPAVPGELTEATPNRYRYYQNVCTQSYSFVWWDWARWEREIDWMALNGINLALAWSGQEAIWQRVYLALGLTQAEINEFFTGPAFLAWGRMGNLHTWDGPLPPSWHIKQLYLQHRVLDQMRSFGMTPVLPAFAGHVPEAVTRVFPQVNVTKMGSWGHFNCSYSCSFLLAPEDPIFPIIGSLFLRELIKEFGTDHIYGADTFNEMQPPSSEPSYLAAATTAVYEAMTAVDPDAVWLLQGWLFQHQPQFWGPAQIRAVLGAVPRGRLLVLDLFAESQPVYTRTASFQGQPFIWCMLHNFGGNHGLFGALEAVNGGPEAARLFPNSTMVGTGMAPEGISQNEVVYSLMAELGWRKDPVPDLAAWVTSFAARRYGVSHPDAGAAWRLLLRSVYNCSGEACRGHNRSPLVRRPSLQMNTSIWYNRSDVFEAWRLLLTSAPSLATSPAFRYDLLDLTRQAVQELVSLYYEEARSAYLSKELASLLRAGGVLAYELLPALDEVLASDSRFLLGSWLEQARAAAVSEAEADFYEQNSRYQLTLWGPEGNILDYANKQLAGLVANYYTPRWRLFLEALVDSVAQGIPFQQHQFDKNVFQLEQAFVLSKQRYPSQPRGDTVDLAKKIFLKYYPRWVAGSW

SEQ ID NO: 16 - DNA, 2229 bp, Artificial Sequence
  nucleic acid sequence coding hNAGLU mutant type 5, synthetic sequence
atggaggctgtggccgtcgccgccgctgtgggcgtgctgctgctggctggcgctggcggcgccgccggcgacgaggctagggaagccgccgccgtgcgggccctcgtggctaggctgctgggccccggtcccgctgccgatttttccgtgagcgtcgagagggccctcgctgctaagcccggtttagacacctactccctcggcggaggaggagctgctagggttcgtgttcgtggatccactggtgtggccgctgctgctggactccatcgttatttacgggatttctgtggatgccacgtggcttggagcggcagccaactgaggctccctaggcctctgcccgctgtccccggtgaactgaccgaggctacccccaatcggtaccggtactaccagaacgtgtgcacccaaagctattccttcgtgtggtgggactgggctcgttgggaaagggagatcgactggatggccctcaacggaattaatctggctttagcttggtccggccaagaggccatttggcagagggtgtacctcgctttaggtttaacacaagctgagatcaacgaattcttcaccggccccgcttttctcgcttggggacggatgggcaatttacacacttgggatggccctctccccccttcttggcacattaagcaactgtatttacagcatcgtgtgctcgatcagatgaggtccttcggcatgacacccgtgctccccgcttttgctggccacgtccccgaagctgtcactcgtgtgtttcctcaagttaacgtgacaaagatgggctcttggggccactttaactgcagctacagctgttcctttttactggcccccgaggatcccatttttcccatcatcggctccctctttttaagggagctgatcaaagagttcggcaccgaccacatttacggcgccgacacctttaacgagatgcagccccctagcagcgagcctagctatttagctgctgccaccacagccgtctatgaggccatgaccgccgtggaccccgacgctgtgtggctgctgcaaggttggctgttccagcaccagcctcagttctggggccccgctcaaattcgtgccgtgctgggcgccgtgcctcggggtcgtctgctggtcctcgatctgttcgctgagtcccaacccgtttacacaaggacagcctccttccaaggtcagcccttcatctggtgcatgctgcacaactttggcggaaaccacggactgttcggagctttagaggctgtgaatggcggacccgaagctgcccggctgttccccaactccaccatggtgggaaccggaatggcccccgaaggcatttcccagaatgaggtggtctacagcctcatggccgagctcggatggcggaaggatcccgttcccgatttagctgcttgggtgacctccttcgctgctcggaggtatggcgtgtcccatcccgatgccggagctgcttggaggttattattacgttccgtctacaactgctccggcgaggcttgccggggacataatcggtcccctttagttcgtaggccttctttacagatgaataccagcatctggtacaaccggagcgacgtgttcgaagcttggcgtttattactgacatccgctccctctttagctaccagccccgcctttcgttatgatttattagatctgactcgtcaagctgtgcaagaactggtgtctttatactacgaggaagctcggagcgcctatttatccaaagagctggcctctttactgagggctggaggcgtgctggcttatgagctgctccccgctttagatgaggttttagctagcgactctcgttttttactgggatcttggctggagcaagctcgtgccgctgccgtgagcgaagccgaggccgatttctatgagcagaactcccggtaccagctgacactctggggccccgagggcaacattctggactacgccaacaagcagctggctggactggtggccaactactacacccctcgttggaggctgtttttagaagctctggtcgactccgtggcccaaggtatccccttccaacagcaccagttcgacaagaatgtgttccagctggaacaagctttcgtgctgtccaaacaaaggtacccctcccagccccggggagacacagtggatctggccaagaagatctttttaaagtattaccctcggtgggtggctggaagctgg

SEQ ID NO: 17 - protein, 720 aa, Artificial Sequence
  amino acid sequence of  hNAGLU mutant type 6
DEAREAAAVRALVARLLGPGPAADFSVSVERALAAKPGLDTYSLGGGGAARVRVRGSTGVAAAAGLHRYLRDFCGCHVAWSGSQLRLPRPLPAVPGELTEATPNRYRYYQNVCTQSYSFVWWDWARWEREIDWMALNGINLALAWSGQEAIWQRVYLALGLTQAEINEFFTGPAFLAWGRMGNLHTWDGPLPPSWHIKQLYLQHRVLDQMRSFGMTPVLPAFAGHVPEAVTRVFPQVNVTKMGSWGHFNCSYSCSFLLAPEDPIFPIIGSLFLRELIKEFGTDHIYGADTFNEMQPPSSEPSYLAAATTAVYEAMTAVDTEAVWLLQGWLFQHQPQFWGPAQIRAVLGAVPRGRLLVLDLFAESQPVYTRTASFQGQPFIWCMLHNFGGNHGLFGALEAVNGGPEAARLFPNSTMVGTGMAPEGISQNEVVYSLMAELGWRKDPVPDLAAWVTSFAARRYGVSHPDAGAAWRLLLRSVYNCSGEACRGHNRSPLVRRPSLQMNTAVWYNRSDVFEAWRLLLTSAPSLATSPAFRYDLLDLTRQAVQELVSLYYEEARSAYLSKELASLLRAGGVLAYELLPALDEVLASDSRFLLGSWLEQARAAAVSEAEADFYEQNSRYQLTLWGPEGNILDYANKQLAGLVANYYTPRWRLFLEALVDSVAQGIPFQQHQFDKNVFQLEQAFVLSKQRYPSQPRGDTVDLAKKIFLKYYPRWVAGSW

SEQ ID NO: 18 - DNA, 2229 bp, Artificial Sequence
  nucleic acid sequence coding hNAGLU mutant type 6, synthetic sequence
atggaggctgtggccgtcgccgccgctgtgggcgtgctgctgctggctggcgctggcggcgccgccggcgacgaggctagggaagccgccgccgtgcgggccctcgtggctaggctgctgggccccggtcccgctgccgatttttccgtgagcgtcgagagggccctcgctgctaagcccggtttagacacctactccctcggcggaggaggagctgctagggttcgtgttcgtggatccactggtgtggccgctgctgctggactccatcgttatttacgggatttctgtggatgccacgtggcttggagcggcagccaactgaggctccctaggcctctgcccgctgtccccggtgaactgaccgaggctacccccaatcggtaccggtactaccagaacgtgtgcacccaaagctattccttcgtgtggtgggactgggctcgttgggaaagggagatcgactggatggccctcaacggaattaatctggctttagcttggtccggccaagaggccatttggcagagggtgtacctcgctttaggtttaacacaagctgagatcaacgaattcttcaccggccccgcttttctcgcttggggacggatgggcaatttacacacttgggatggccctctccccccttcttggcacattaagcaactgtatttacagcatcgtgtgctcgatcagatgaggtccttcggcatgacacccgtgctccccgcttttgctggccacgtccccgaagctgtcactcgtgtgtttcctcaagttaacgtgacaaagatgggctcttggggccactttaactgcagctacagctgttcctttttactggcccccgaggatcccatttttcccatcatcggctccctctttttaagggagctgatcaaagagttcggcaccgaccacatttacggcgccgacacctttaacgagatgcagccccctagcagcgagcctagctatttagctgctgccaccacagccgtctatgaggccatgaccgccgtggacaccgaagctgtgtggctgctgcaaggttggctgttccagcaccagcctcagttctggggccccgctcaaattcgtgccgtgctgggcgccgtgcctcggggtcgtctgctggtcctcgatctgttcgctgagtcccaacccgtttacacaaggacagcctccttccaaggtcagcccttcatctggtgcatgctgcacaactttggcggaaaccacggactgttcggagctttagaggctgtgaatggcggacccgaagctgcccggctgttccccaactccaccatggtgggaaccggaatggcccccgaaggcatttcccagaatgaggtggtctacagcctcatggccgagctcggatggcggaaggatcccgttcccgatttagctgcttgggtgacctccttcgctgctcggaggtatggcgtgtcccatcccgatgccggagctgcttggaggttattattacgttccgtctacaactgctccggcgaggcttgccggggacataatcggtcccctttagttcgtaggccttctttacagatgaataccgccgtctggtacaaccggagcgacgtgttcgaagcttggcgtttattactgacatccgctccctctttagctaccagccccgcctttcgttatgatttattagatctgactcgtcaagctgtgcaagaactggtgtctttatactacgaggaagctcggagcgcctatttatccaaagagctggcctctttactgagggctggaggcgtgctggcttatgagctgctccccgctttagatgaggttttagctagcgactctcgttttttactgggatcttggctggagcaagctcgtgccgctgccgtgagcgaagccgaggccgatttctatgagcagaactcccggtaccagctgacactctggggccccgagggcaacattctggactacgccaacaagcagctggctggactggtggccaactactacacccctcgttggaggctgtttttagaagctctggtcgactccgtggcccaaggtatccccttccaacagcaccagttcgacaagaatgtgttccagctggaacaagctttcgtgctgtccaaacaaaggtacccctcccagccccggggagacacagtggatctggccaagaagatctttttaaagtattaccctcggtgggtggctggaagctgg

SEQ ID NO: 19 - protein, 720 aa, Artificial Sequence
  amino acid sequence of  hNAGLU mutant type 7
DEAREAAAVRALVARLLGPGPAADFSVSVERALAAKPGLDTYSLGGGGAARVRVRGSTGVAAAAGLHRYLRDFCGCHVAWSGSQLRLPRPLPAVPGELTEATPNRYRYYQNVCTQSYSFVWWDWARWEREIDWMALNGINLALAWSGQEAIWQRVYLALGLTQAEINEFFTGPAFLAWGRMGNLHTWDGPLPPSWHIKQLYLQHRVLDQMRSFGMTPVLPAFAGHVPEAVTRVFPQVNVTKMGSWGHFNCSYSCSFLLAPEDPIFPIIGSLFLRELIKEFGTDHIYGADTFNEMQPPSSEPSYLAAATTAVYEAMTAVDTEAVWLLQGWLFQHQPQFWGPAQIRAVLGAVPRGRLLVLDLFAESQPVYTRTASFQGQPFIWCMLHNFGGNHGLFGALEAVNGGPEAARLFPNSTMVGTGMAPEGISQNEVVYSLMAELGWRKDPVPDLAAWVTSFAARRYGVSHPDAGAAWRLLLRSVYNCSGEACRGHNRSPLVRRPSLQMNTSIWYNRSDVFEAWRLLLTSAPNLTTSPAFRYDLLDLTRQAVQELVSLYYEEARSAYLSKELASLLRAGGVLAYELLPALDEVLASDSRFLLGSWLEQARAAAVSEAEADFYEQNSRYQLTLWGPEGNILDYANKQLAGLVANYYTPRWRLFLEALVDSVAQGIPFQQHQFDKNVFQLEQAFVLSKQRYPSQPRGDTVDLAKKIFLKYYPRWVAGSW

SEQ ID NO: 20 - DNA, 2229 bp, Artificial Sequence
  nucleic acid sequence coding hNAGLU mutant type 7, synthetic sequence
atggaggctgtggccgtcgccgccgctgtgggcgtgctgctgctggctggcgctggcggcgccgccggcgacgaggctagggaagccgccgccgtgcgggccctcgtggctaggctgctgggccccggtcccgctgccgatttttccgtgagcgtcgagagggccctcgctgctaagcccggtttagacacctactccctcggcggaggaggagctgctagggttcgtgttcgtggatccactggtgtggccgctgctgctggactccatcgttatttacgggatttctgtggatgccacgtggcttggagcggcagccaactgaggctccctaggcctctgcccgctgtccccggtgaactgaccgaggctacccccaatcggtaccggtactaccagaacgtgtgcacccaaagctattccttcgtgtggtgggactgggctcgttgggaaagggagatcgactggatggccctcaacggaattaatctggctttagcttggtccggccaagaggccatttggcagagggtgtacctcgctttaggtttaacacaagctgagatcaacgaattcttcaccggccccgcttttctcgcttggggacggatgggcaatttacacacttgggatggccctctccccccttcttggcacattaagcaactgtatttacagcatcgtgtgctcgatcagatgaggtccttcggcatgacacccgtgctccccgcttttgctggccacgtccccgaagctgtcactcgtgtgtttcctcaagttaacgtgacaaagatgggctcttggggccactttaactgcagctacagctgttcctttttactggcccccgaggatcccatttttcccatcatcggctccctctttttaagggagctgatcaaagagttcggcaccgaccacatttacggcgccgacacctttaacgagatgcagccccctagcagcgagcctagctatttagctgctgccaccacagccgtctatgaggccatgaccgccgtggacaccgaagctgtgtggctgctgcaaggttggctgttccagcaccagcctcagttctggggccccgctcaaattcgtgccgtgctgggcgccgtgcctcggggtcgtctgctggtcctcgatctgttcgctgagtcccaacccgtttacacaaggacagcctccttccaaggtcagcccttcatctggtgcatgctgcacaactttggcggaaaccacggactgttcggagctttagaggctgtgaatggcggacccgaagctgcccggctgttccccaactccaccatggtgggaaccggaatggcccccgaaggcatttcccagaatgaggtggtctacagcctcatggccgagctcggatggcggaaggatcccgttcccgatttagctgcttgggtgacctccttcgctgctcggaggtatggcgtgtcccatcccgatgccggagctgcttggaggttattattacgttccgtctacaactgctccggcgaggcttgccggggacataatcggtcccctttagttcgtaggccttctttacagatgaataccagcatctggtacaaccggagcgacgtgttcgaagcttggcgtttattactgacatccgctcccaatttaactaccagccccgcctttcgttatgatttattagatctgactcgtcaagctgtgcaagaactggtgtctttatactacgaggaagctcggagcgcctatttatccaaagagctggcctctttactgagggctggaggcgtgctggcttatgagctgctccccgctttagatgaggttttagctagcgactctcgttttttactgggatcttggctggagcaagctcgtgccgctgccgtgagcgaagccgaggccgatttctatgagcagaactcccggtaccagctgacactctggggccccgagggcaacattctggactacgccaacaagcagctggctggactggtggccaactactacacccctcgttggaggctgtttttagaagctctggtcgactccgtggcccaaggtatccccttccaacagcaccagttcgacaagaatgtgttccagctggaacaagctttcgtgctgtccaaacaaaggtacccctcccagccccggggagacacagtggatctggccaagaagatctttttaaagtattaccctcggtgggtggctggaagctgg

SEQ ID NO: 21 - protein, 720 aa, Artificial Sequence
  amino acid sequence of  hNAGLU mutant type 18
DEAREAAAVRALVARLLGPGPAADFSVSVERALAAKPGLDTYSLGGGGAARVRVRGSTGVAAAAGLHRYLRDFCGCHVAWSGSQLRLPRPLPAVPGELTEATPNRYRYYQNVCTQSYSFVWWDWARWEREIDWMALNGINLALAWSGQEAIWQRVYLALGLTQAEINEFFTGPAFLAWGRMGNLHTWDGPLPPSWHIKQLYLQHRVLDQMRSFGMTPVLPAFAGHVPEAVTRVFPQVNVTKMGSWGHFNCSYSCSFLLAPEDPIFPIIGSLFLRELIKEFGTDHIYGADTFNEMQPPSSEPSYLAAATTAVYEAMTAVDTEAVWLLQGWLFQHQPQFWGPAQIRAVLGAVPRGRLLVLDLFAESQPVYTRTASFQGQPFIWCMLHNFGGNHGLFGALEAVNGGPEAARLFPNSTMVGTGMAPEGISQNEVVYSLMAELGWRKDPVPDLAAWVTSFAARRYGVSHPDAGAAWRLLLRSVYNCSGEACRGHNRSPLVRRPSLQMNTSIWYNRSDVFEAWRLLLTSAPSLATSPAFRYDLLDLTRQAVQELVSLYYEEARSAYLSKELASLLRAGGVLAYELLPALDEVLASDSRFLLGSWLEQARAAAVSEAEAQFYEQNSRYQLTLWGPEGNILDYANKQLAGLVANYYTPRWRLFLEALVDSVAQGIPFQQHQFDKNVFQLEQAFVLSKQRYPSQPRGDTVDLAKKIFLKYYPRWVAGSW

SEQ ID NO: 22 - DNA, 2229 bp, Artificial Sequence
  nucleic acid sequence coding hNAGLU mutant type 18, synthetic sequence
atggaggctgtggccgtcgccgccgctgtgggcgtgctgctgctggctggcgctggcggcgccgccggcgacgaggctagggaagccgccgccgtgcgggccctcgtggctaggctgctgggccccggtcccgctgccgatttttccgtgagcgtcgagagggccctcgctgctaagcccggtttagacacctactccctcggcggaggaggagctgctagggttcgtgttcgtggatccactggtgtggccgctgctgctggactccatcgttatttacgggatttctgtggatgccacgtggcttggagcggcagccaactgaggctccctaggcctctgcccgctgtccccggtgaactgaccgaggctacccccaatcggtaccggtactaccagaacgtgtgcacccaaagctattccttcgtgtggtgggactgggctcgttgggaaagggagatcgactggatggccctcaacggaattaatctggctttagcttggtccggccaagaggccatttggcagagggtgtacctcgctttaggtttaacacaagctgagatcaacgaattcttcaccggccccgcttttctcgcttggggacggatgggcaatttacacacttgggatggccctctccccccttcttggcacattaagcaactgtatttacagcatcgtgtgctcgatcagatgaggtccttcggcatgacacccgtgctccccgcttttgctggccacgtccccgaagctgtcactcgtgtgtttcctcaagttaacgtgacaaagatgggctcttggggccactttaactgcagctacagctgttcctttttactggcccccgaggatcccatttttcccatcatcggctccctctttttaagggagctgatcaaagagttcggcaccgaccacatttacggcgccgacacctttaacgagatgcagccccctagcagcgagcctagctatttagctgctgccaccacagccgtctatgaggccatgaccgccgtggacaccgaagctgtgtggctgctgcaaggttggctgttccagcaccagcctcagttctggggccccgctcaaattcgtgccgtgctgggcgccgtgcctcggggtcgtctgctggtcctcgatctgttcgctgagtcccaacccgtttacacaaggacagcctccttccaaggtcagcccttcatctggtgcatgctgcacaactttggcggaaaccacggactgttcggagctttagaggctgtgaatggcggacccgaagctgcccggctgttccccaactccaccatggtgggaaccggaatggcccccgaaggcatttcccagaatgaggtggtctacagcctcatggccgagctcggatggcggaaggatcccgttcccgatttagctgcttgggtgacctccttcgctgctcggaggtatggcgtgtcccatcccgatgccggagctgcttggaggttattattacgttccgtctacaactgctccggcgaggcttgccggggacataatcggtcccctttagttcgtaggccttctttacagatgaataccagcatctggtacaaccggagcgacgtgttcgaagcttggcgtttattactgacatccgctccctctttagctaccagccccgcctttcgttatgatttattagatctgactcgtcaagctgtgcaagaactggtgtctttatactacgaggaagctcggagcgcctatttatccaaagagctggcctctttactgagggctggaggcgtgctggcttatgagctgctccccgctttagatgaggttttagctagcgactctcgttttttactgggatcttggctggagcaagctcgtgccgctgccgtgagcgaagccgaggcccagttctatgagcagaactcccggtaccagctgacactctggggccccgagggcaacattctggactacgccaacaagcagctggctggactggtggccaactactacacccctcgttggaggctgtttttagaagctctggtcgactccgtggcccaaggtatccccttccaacagcaccagttcgacaagaatgtgttccagctggaacaagctttcgtgctgtccaaacaaaggtacccctcccagccccggggagacacagtggatctggccaagaagatctttttaaagtattaccctcggtgggtggctggaagctgg

SEQ ID NO: 23 - protein, 720 aa, Artificial Sequence
  amino acid sequence of  hNAGLU mutant type 19
DEAREAAAVRALVARLLGPGPAADFSVSVERALAAKPGLDTYSLGGGGAARVRVRGSTGVAAAAGLHRYLRDFCGCHVAWSGSQLRLPRPLPAVPGELTEATPNRYRYYQNVCTQSYSFVWWDWARWEREIDWMALNGINLALAWSGQEAIWQRVYLALGLTQAEINEFFTGPAFLAWGRMGNLHTWDGPLPPSWHIKQLYLQKRVLDQMRSFGMTPVLPAFAGHVPEAVTRVFPQVNVTKMGSWGHFNCSYSCSFLLAPEDPIFPIIGSLFLRELIKEFGTDHIYGADTFNEMQPPSSEPSYLAAATTAVYEAMTAVDTEAVWLLQGWLFQHQPQFWGPAQIRAVLGAVPRGRLLVLDLFAESQPVYTRTASFQGQPFIWCMLHNFGGNHGLFGALEAVNGGPEAARLFPNSTMVGTGMAPEGISQNEVVYSLMAELGWRKDPVPDLAAWVTSFAARRYGVSHPDAGAAWRLLLRSVYNCSGEACRGHNRSPLVRRPSLQMNTSIWYNRSDVFEAWRLLLTSAPSLATSPAFRYDLLDLTRQAVQELVSLYYEEARSAYLSKELASLLRAGGVLAYELLPALDEVLASDSRFLLGSWLEQARAAAVSEAEADFYEQNSRYQLTLWGPEGNILDYANKQLAGLVANYYTPRWRLFLEALVDSVAQGIPFQQHQFDKNVFQLEQAFVLSKQRYPSQPRGDTVDLAKKIFLKYYPRWVAGSW

SEQ ID NO: 24 - DNA, 2229 bp, Artificial Sequence
  nucleic acid sequence coding hNAGLU mutant type 19, synthetic sequence
atggaggctgtggccgtcgccgccgctgtgggcgtgctgctgctggctggcgctggcggcgccgccggcgacgaggctagggaagccgccgccgtgcgggccctcgtggctaggctgctgggccccggtcccgctgccgatttttccgtgagcgtcgagagggccctcgctgctaagcccggtttagacacctactccctcggcggaggaggagctgctagggttcgtgttcgtggatccactggtgtggccgctgctgctggactccatcgttatttacgggatttctgtggatgccacgtggcttggagcggcagccaactgaggctccctaggcctctgcccgctgtccccggtgaactgaccgaggctacccccaatcggtaccggtactaccagaacgtgtgcacccaaagctattccttcgtgtggtgggactgggctcgttgggaaagggagatcgactggatggccctcaacggaattaatctggctttagcttggtccggccaagaggccatttggcagagggtgtacctcgctttaggtttaacacaagctgagatcaacgaattcttcaccggccccgcttttctcgcttggggacggatgggcaatttacacacttgggatggccctctccccccttcttggcacattaagcaactgtatttacagaagcgtgtgctcgatcagatgaggtccttcggcatgacacccgtgctccccgcttttgctggccacgtccccgaagctgtcactcgtgtgtttcctcaagttaacgtgacaaagatgggctcttggggccactttaactgcagctacagctgttcctttttactggcccccgaggatcccatttttcccatcatcggctccctctttttaagggagctgatcaaagagttcggcaccgaccacatttacggcgccgacacctttaacgagatgcagccccctagcagcgagcctagctatttagctgctgccaccacagccgtctatgaggccatgaccgccgtggacaccgaagctgtgtggctgctgcaaggttggctgttccagcaccagcctcagttctggggccccgctcaaattcgtgccgtgctgggcgccgtgcctcggggtcgtctgctggtcctcgatctgttcgctgagtcccaacccgtttacacaaggacagcctccttccaaggtcagcccttcatctggtgcatgctgcacaactttggcggaaaccacggactgttcggagctttagaggctgtgaatggcggacccgaagctgcccggctgttccccaactccaccatggtgggaaccggaatggcccccgaaggcatttcccagaatgaggtggtctacagcctcatggccgagctcggatggcggaaggatcccgttcccgatttagctgcttgggtgacctccttcgctgctcggaggtatggcgtgtcccatcccgatgccggagctgcttggaggttattattacgttccgtctacaactgctccggcgaggcttgccggggacataatcggtcccctttagttcgtaggccttctttacagatgaataccagcatctggtacaaccggagcgacgtgttcgaagcttggcgtttattactgacatccgctccctctttagctaccagccccgcctttcgttatgatttattagatctgactcgtcaagctgtgcaagaactggtgtctttatactacgaggaagctcggagcgcctatttatccaaagagctggcctctttactgagggctggaggcgtgctggcttatgagctgctccccgctttagatgaggttttagctagcgactctcgttttttactgggatcttggctggagcaagctcgtgccgctgccgtgagcgaagccgaggccgatttctatgagcagaactcccggtaccagctgacactctggggccccgagggcaacattctggactacgccaacaagcagctggctggactggtggccaactactacacccctcgttggaggctgtttttagaagctctggtcgactccgtggcccaaggtatccccttccaacagcaccagttcgacaagaatgtgttccagctggaacaagctttcgtgctgtccaaacaaaggtacccctcccagccccggggagacacagtggatctggccaagaagatctttttaaagtattaccctcggtgggtggctggaagctgg

SEQ ID NO: 25 - protein, 720 aa, Artificial Sequence
  amino acid sequence of  hNAGLU mutant type 8
DEAREAAAVRALVARLLGPGPAADFSVSVERALAAESGLDTYSLGGGGAARVRVRGSTGVAAAAGLHRYLRDFCGCHVAWSGSQLRLPRPLPAVPGELTEATPNRYRYYQNVCTQSYSFVWWDWARWEREIDWMALNGINLALAWSGQEAIWQRVYLALGLTQAEINEFFTGPAFLAWGRMGNLHTWDGPLPPSWHIKQLYLQHRVLDRMRSFGMTPVLPAFAGHVPEAVTRVFPQVNVTKMGSWGHFNCSYSCSFLLAPEDPIFPIIGSLFLRELIKEFGTDHIYGADTFNEMQPPSSEPSYLAAATTAVYEAMTAVDTEAVWLLQGWLFQHQPQFWGPAQIRAVLGAVPRGRLLVLDLFAESQPVYTRTASFQGQPFIWCMLHNFGGNHGLFGALEAVNGGPEAARLFPNSTMVGTGMAPEGISQNEVVYSLMAELGWRKDPVPDLAAWVTSFAARRYGVSHPDAGAAWRLLLRSVYNCSGEACRGHNRSPLVRRPSLQMNTSIWYNRSDVFEAWRLLLTSAPSLATSPAFRYDLLDLTRQAVQELVSLYYEEARSAYLSKELASLLRAGGVLAYELLPALDEVLASDSRFLLGSWLEQARAAAVSEAEADFYEQNSRYQLTLWGPEGNILDYANKQLAGLVANYYTPRWRLFLEALVDSVAQGIPFQQHQFDKNVFQLEQAFVLSKQRYPSQPRGDTVDLAKKIFLKYYPRWVAGSW

SEQ ID NO: 26 - DNA, 2229 bp, Artificial Sequence
  nucleic acid sequence coding hNAGLU mutant type 8, synthetic sequence
atggaggctgtggccgtcgccgccgctgtgggcgtgctgctgctggctggcgctggcggcgccgccggcgacgaggctagggaagccgccgccgtgcgggccctcgtggctaggctgctgggccccggtcccgctgccgatttttccgtgagcgtcgagagggccctcgctgctgagtccggtttagacacctactccctcggcggaggaggagctgctagggttcgtgttcgtggatccactggtgtggccgctgctgctggactccatcgttatttacgggatttctgtggatgccacgtggcttggagcggcagccaactgaggctccctaggcctctgcccgctgtccccggtgaactgaccgaggctacccccaatcggtaccggtactaccagaacgtgtgcacccaaagctattccttcgtgtggtgggactgggctcgttgggaaagggagatcgactggatggccctcaacggaattaatctggctttagcttggtccggccaagaggccatttggcagagggtgtacctcgctttaggtttaacacaagctgagatcaacgaattcttcaccggccccgcttttctcgcttggggacggatgggcaatttacacacttgggatggccctctccccccttcttggcacattaagcaactgtatttacagcatcgtgtgctcgatcggatgaggtccttcggcatgacacccgtgctccccgcttttgctggccacgtccccgaagctgtcactcgtgtgtttcctcaagttaacgtgacaaagatgggctcttggggccactttaactgcagctacagctgttcctttttactggcccccgaggatcccatttttcccatcatcggctccctctttttaagggagctgatcaaagagttcggcaccgaccacatttacggcgccgacacctttaacgagatgcagccccctagcagcgagcctagctatttagctgctgccaccacagccgtctatgaggccatgaccgccgtggacaccgaagctgtgtggctgctgcaaggttggctgttccagcaccagcctcagttctggggccccgctcaaattcgtgccgtgctgggcgccgtgcctcggggtcgtctgctggtcctcgatctgttcgctgagtcccaacccgtttacacaaggacagcctccttccaaggtcagcccttcatctggtgcatgctgcacaactttggcggaaaccacggactgttcggagctttagaggctgtgaatggcggacccgaagctgcccggctgttccccaactccaccatggtgggaaccggaatggcccccgaaggcatttcccagaatgaggtggtctacagcctcatggccgagctcggatggcggaaggatcccgttcccgatttagctgcttgggtgacctccttcgctgctcggaggtatggcgtgtcccatcccgatgccggagctgcttggaggttattattacgttccgtctacaactgctccggcgaggcttgccggggacataatcggtcccctttagttcgtaggccttctttacagatgaataccagcatctggtacaaccggagcgacgtgttcgaagcttggcgtttattactgacatccgctccctctttagctaccagccccgcctttcgttatgatttattagatctgactcgtcaagctgtgcaagaactggtgtctttatactacgaggaagctcggagcgcctatttatccaaagagctggcctctttactgagggctggaggcgtgctggcttatgagctgctccccgctttagatgaggttttagctagcgactctcgttttttactgggatcttggctggagcaagctcgtgccgctgccgtgagcgaagccgaggccgatttctatgagcagaactcccggtaccagctgacactctggggccccgagggcaacattctggactacgccaacaagcagctggctggactggtggccaactactacacccctcgttggaggctgtttttagaagctctggtcgactccgtggcccaaggtatccccttccaacagcaccagttcgacaagaatgtgttccagctggaacaagctttcgtgctgtccaaacaaaggtacccctcccagccccggggagacacagtggatctggccaagaagatctttttaaagtattaccctcggtgggtggctggaagctgg

SEQ ID NO: 27 - protein, 721 aa, Artificial Sequence
  amino acid sequence of  hNAGLU mutant type 9
DEAREAAAVRALVARLLGPGPAADFSVSVERALAAKPGLDTYSLSGGGGAARVRVRGSTGVAAAAGLHRYLRDFCGCHVAWSGSQLRLPRPLPAVPGELTEATPNRYRYYQNVCTQSYSFVWWDWARWEREIDWMALNGINLALAWSGQEAIWQRVYLALGLTQAEINEFFTGPAFLAWGRMGNLHTWDGPLPPSWHIKQLYLQHRVLDRMRSFGMTPVLPAFAGHVPEAVTRVFPQVNVTKMGSWGHFNCSYSCSFLLAPEDPIFPIIGSLFLRELIKEFGTDHIYGADTFNEMQPPSSEPSYLAAATTAVYEAMTAVDTEAVWLLQGWLFQHQPQFWGPAQIRAVLGAVPRGRLLVLDLFAESQPVYTRTASFQGQPFIWCMLHNFGGNHGLFGALEAVNGGPEAARLFPNSTMVGTGMAPEGISQNEVVYSLMAELGWRKDPVPDLAAWVTSFAARRYGVSHPDAGAAWRLLLRSVYNCSGEACRGHNRSPLVRRPSLQMNTSIWYNRSDVFEAWRLLLTSAPSLATSPAFRYDLLDLTRQAVQELVSLYYEEARSAYLSKELASLLRAGGVLAYELLPALDEVLASDSRFLLGSWLEQARAAAVSEAEADFYEQNSRYQLTLWGPEGNILDYANKQLAGLVANYYTPRWRLFLEALVDSVAQGIPFQQHQFDKNVFQLEQAFVLSKQRYPSQPRGDTVDLAKKIFLKYYPRWVAGSW

SEQ ID NO: 28 - DNA, 2232 bp, Artificial Sequence
  nucleic acid sequence coding hNAGLU mutant type 9, synthetic sequence
atggaggctgtggccgtcgccgccgctgtgggcgtgctgctgctggctggcgctggcggcgccgccggcgacgaggctagggaagccgccgccgtgcgggccctcgtggctaggctgctgggccccggtcccgctgccgatttttccgtgagcgtcgagagggccctcgctgctaagcccggtttagacacctactccctctctggcggaggaggagctgctagggttcgtgttcgtggatccactggtgtggccgctgctgctggactccatcgttatttacgggatttctgtggatgccacgtggcttggagcggcagccaactgaggctccctaggcctctgcccgctgtccccggtgaactgaccgaggctacccccaatcggtaccggtactaccagaacgtgtgcacccaaagctattccttcgtgtggtgggactgggctcgttgggaaagggagatcgactggatggccctcaacggaattaatctggctttagcttggtccggccaagaggccatttggcagagggtgtacctcgctttaggtttaacacaagctgagatcaacgaattcttcaccggccccgcttttctcgcttggggacggatgggcaatttacacacttgggatggccctctccccccttcttggcacattaagcaactgtatttacagcatcgtgtgctcgatcggatgaggtccttcggcatgacacccgtgctccccgcttttgctggccacgtccccgaagctgtcactcgtgtgtttcctcaagttaacgtgacaaagatgggctcttggggccactttaactgcagctacagctgttcctttttactggcccccgaggatcccatttttcccatcatcggctccctctttttaagggagctgatcaaagagttcggcaccgaccacatttacggcgccgacacctttaacgagatgcagccccctagcagcgagcctagctatttagctgctgccaccacagccgtctatgaggccatgaccgccgtggacaccgaagctgtgtggctgctgcaaggttggctgttccagcaccagcctcagttctggggccccgctcaaattcgtgccgtgctgggcgccgtgcctcggggtcgtctgctggtcctcgatctgttcgctgagtcccaacccgtttacacaaggacagcctccttccaaggtcagcccttcatctggtgcatgctgcacaactttggcggaaaccacggactgttcggagctttagaggctgtgaatggcggacccgaagctgcccggctgttccccaactccaccatggtgggaaccggaatggcccccgaaggcatttcccagaatgaggtggtctacagcctcatggccgagctcggatggcggaaggatcccgttcccgatttagctgcttgggtgacctccttcgctgctcggaggtatggcgtgtcccatcccgatgccggagctgcttggaggttattattacgttccgtctacaactgctccggcgaggcttgccggggacataatcggtcccctttagttcgtaggccttctttacagatgaataccagcatctggtacaaccggagcgacgtgttcgaagcttggcgtttattactgacatccgctccctctttagctaccagccccgcctttcgttatgatttattagatctgactcgtcaagctgtgcaagaactggtgtctttatactacgaggaagctcggagcgcctatttatccaaagagctggcctctttactgagggctggaggcgtgctggcttatgagctgctccccgctttagatgaggttttagctagcgactctcgttttttactgggatcttggctggagcaagctcgtgccgctgccgtgagcgaagccgaggccgatttctatgagcagaactcccggtaccagctgacactctggggccccgagggcaacattctggactacgccaacaagcagctggctggactggtggccaactactacacccctcgttggaggctgtttttagaagctctggtcgactccgtggcccaaggtatccccttccaacagcaccagttcgacaagaatgtgttccagctggaacaagctttcgtgctgtccaaacaaaggtacccctcccagccccggggagacacagtggatctggccaagaagatctttttaaagtattaccctcggtgggtggctggaagctgg

SEQ ID NO: 29 - protein, 720 aa, Artificial Sequence
  amino acid sequence of  hNAGLU mutant type 10
DEAREAAAVRALVARLLGPGPAADFSVSVERALAAKPGLDTYSLGGGGAARVRVRGSTGVAAAAGLHRYLRDFCGCHVAWSGSQLRLPRPLPAVPGELTEATPNRYRYYQNVCTQSYSFVWWDWARWEREIDWMALNGINLALAWSGQEAIWQRVYLALGLTQAEINEFFTGPAFLAWGRMGNLHTWDGPLPPSWHIKQLYLQHRVLDRMRSFGMTPVLPAFAGHVPEAVTRVFPQVNVTKMGSWGHFNCSYSCSFLLAPEDPIFPIIGSLFLRELIKEFGTDHIYGADTFNEMQPPSSEPSYLAAATTAVYEAMTAVDPDAVWLLQGWLFQHQPQFWGPAQIRAVLGAVPRGRLLVLDLFAESQPVYTRTASFQGQPFIWCMLHNFGGNHGLFGALEAVNGGPEAARLFPNSTMVGTGMAPEGISQNEVVYSLMAELGWRKDPVPDLAAWVTSFAARRYGVSHPDAGAAWRLLLRSVYNCSGEACRGHNRSPLVRRPSLQMNTSIWYNRSDVFEAWRLLLTSAPSLATSPAFRYDLLDLTRQAVQELVSLYYEEARSAYLSKELASLLRAGGVLAYELLPALDEVLASDSRFLLGSWLEQARAAAVSEAEADFYEQNSRYQLTLWGPEGNILDYANKQLAGLVANYYTPRWRLFLEALVDSVAQGIPFQQHQFDKNVFQLEQAFVLSKQRYPSQPRGDTVDLAKKIFLKYYPRWVAGSW

SEQ ID NO: 30 - DNA, 2229 bp, Artificial Sequence
  nucleic acid sequence coding hNAGLU mutant type 10, synthetic sequence
atggaggctgtggccgtcgccgccgctgtgggcgtgctgctgctggctggcgctggcggcgccgccggcgacgaggctagggaagccgccgccgtgcgggccctcgtggctaggctgctgggccccggtcccgctgccgatttttccgtgagcgtcgagagggccctcgctgctaagcccggtttagacacctactccctcggcggaggaggagctgctagggttcgtgttcgtggatccactggtgtggccgctgctgctggactccatcgttatttacgggatttctgtggatgccacgtggcttggagcggcagccaactgaggctccctaggcctctgcccgctgtccccggtgaactgaccgaggctacccccaatcggtaccggtactaccagaacgtgtgcacccaaagctattccttcgtgtggtgggactgggctcgttgggaaagggagatcgactggatggccctcaacggaattaatctggctttagcttggtccggccaagaggccatttggcagagggtgtacctcgctttaggtttaacacaagctgagatcaacgaattcttcaccggccccgcttttctcgcttggggacggatgggcaatttacacacttgggatggccctctccccccttcttggcacattaagcaactgtatttacagcatcgtgtgctcgatcggatgaggtccttcggcatgacacccgtgctccccgcttttgctggccacgtccccgaagctgtcactcgtgtgtttcctcaagttaacgtgacaaagatgggctcttggggccactttaactgcagctacagctgttcctttttactggcccccgaggatcccatttttcccatcatcggctccctctttttaagggagctgatcaaagagttcggcaccgaccacatttacggcgccgacacctttaacgagatgcagccccctagcagcgagcctagctatttagctgctgccaccacagccgtctatgaggccatgaccgccgtggaccccgacgctgtgtggctgctgcaaggttggctgttccagcaccagcctcagttctggggccccgctcaaattcgtgccgtgctgggcgccgtgcctcggggtcgtctgctggtcctcgatctgttcgctgagtcccaacccgtttacacaaggacagcctccttccaaggtcagcccttcatctggtgcatgctgcacaactttggcggaaaccacggactgttcggagctttagaggctgtgaatggcggacccgaagctgcccggctgttccccaactccaccatggtgggaaccggaatggcccccgaaggcatttcccagaatgaggtggtctacagcctcatggccgagctcggatggcggaaggatcccgttcccgatttagctgcttgggtgacctccttcgctgctcggaggtatggcgtgtcccatcccgatgccggagctgcttggaggttattattacgttccgtctacaactgctccggcgaggcttgccggggacataatcggtcccctttagttcgtaggccttctttacagatgaataccagcatctggtacaaccggagcgacgtgttcgaagcttggcgtttattactgacatccgctccctctttagctaccagccccgcctttcgttatgatttattagatctgactcgtcaagctgtgcaagaactggtgtctttatactacgaggaagctcggagcgcctatttatccaaagagctggcctctttactgagggctggaggcgtgctggcttatgagctgctccccgctttagatgaggttttagctagcgactctcgttttttactgggatcttggctggagcaagctcgtgccgctgccgtgagcgaagccgaggccgatttctatgagcagaactcccggtaccagctgacactctggggccccgagggcaacattctggactacgccaacaagcagctggctggactggtggccaactactacacccctcgttggaggctgtttttagaagctctggtcgactccgtggcccaaggtatccccttccaacagcaccagttcgacaagaatgtgttccagctggaacaagctttcgtgctgtccaaacaaaggtacccctcccagccccggggagacacagtggatctggccaagaagatctttttaaagtattaccctcggtgggtggctggaagctgg

SEQ ID NO: 31 - protein, 721 aa, Artificial Sequence
  amino acid sequence of  hNAGLU mutant type 11
DEAREAAAVRALVARLLGPGPAADFSVSVERALAAESGLDTYSLSGGGGAARVRVRGSTGVAAAAGLHRYLRDFCGCHVAWSGSQLRLPRPLPAVPGELTEATPNRYRYYQNVCTQSYSFVWWDWARWEREIDWMALNGINLALAWSGQEAIWQRVYLALGLTQAEINEFFTGPAFLAWGRMGNLHTWDGPLPPSWHIKQLYLQHRVLDRMRSFGMTPVLPAFAGHVPEAVTRVFPQVNVTKMGSWGHFNCSYSCSFLLAPEDPIFPIIGSLFLRELIKEFGTDHIYGADTFNEMQPPSSEPSYLAAATTAVYEAMTAVDTEAVWLLQGWLFQHQPQFWGPAQIRAVLGAVPRGRLLVLDLFAESQPVYTRTASFQGQPFIWCMLHNFGGNHGLFGALEAVNGGPEAARLFPNSTMVGTGMAPEGISQNEVVYSLMAELGWRKDPVPDLAAWVTSFAARRYGVSHPDAGAAWRLLLRSVYNCSGEACRGHNRSPLVRRPSLQMNTSIWYNRSDVFEAWRLLLTSAPSLATSPAFRYDLLDLTRQAVQELVSLYYEEARSAYLSKELASLLRAGGVLAYELLPALDEVLASDSRFLLGSWLEQARAAAVSEAEADFYEQNSRYQLTLWGPEGNILDYANKQLAGLVANYYTPRWRLFLEALVDSVAQGIPFQQHQFDKNVFQLEQAFVLSKQRYPSQPRGDTVDLAKKIFLKYYPRWVAGSW

SEQ ID NO: 32 - DNA, 2232 bp, Artificial Sequence
  nucleic acid sequence coding hNAGLU mutant type 11, synthetic sequence
atggaggctgtggccgtcgccgccgctgtgggcgtgctgctgctggctggcgctggcggcgccgccggcgacgaggctagggaagccgccgccgtgcgggccctcgtggctaggctgctgggccccggtcccgctgccgatttttccgtgagcgtcgagagggccctcgctgctgagtccggtttagacacctactccctctctggcggaggaggagctgctagggttcgtgttcgtggatccactggtgtggccgctgctgctggactccatcgttatttacgggatttctgtggatgccacgtggcttggagcggcagccaactgaggctccctaggcctctgcccgctgtccccggtgaactgaccgaggctacccccaatcggtaccggtactaccagaacgtgtgcacccaaagctattccttcgtgtggtgggactgggctcgttgggaaagggagatcgactggatggccctcaacggaattaatctggctttagcttggtccggccaagaggccatttggcagagggtgtacctcgctttaggtttaacacaagctgagatcaacgaattcttcaccggccccgcttttctcgcttggggacggatgggcaatttacacacttgggatggccctctccccccttcttggcacattaagcaactgtatttacagcatcgtgtgctcgatcggatgaggtccttcggcatgacacccgtgctccccgcttttgctggccacgtccccgaagctgtcactcgtgtgtttcctcaagttaacgtgacaaagatgggctcttggggccactttaactgcagctacagctgttcctttttactggcccccgaggatcccatttttcccatcatcggctccctctttttaagggagctgatcaaagagttcggcaccgaccacatttacggcgccgacacctttaacgagatgcagccccctagcagcgagcctagctatttagctgctgccaccacagccgtctatgaggccatgaccgccgtggacaccgaagctgtgtggctgctgcaaggttggctgttccagcaccagcctcagttctggggccccgctcaaattcgtgccgtgctgggcgccgtgcctcggggtcgtctgctggtcctcgatctgttcgctgagtcccaacccgtttacacaaggacagcctccttccaaggtcagcccttcatctggtgcatgctgcacaactttggcggaaaccacggactgttcggagctttagaggctgtgaatggcggacccgaagctgcccggctgttccccaactccaccatggtgggaaccggaatggcccccgaaggcatttcccagaatgaggtggtctacagcctcatggccgagctcggatggcggaaggatcccgttcccgatttagctgcttgggtgacctccttcgctgctcggaggtatggcgtgtcccatcccgatgccggagctgcttggaggttattattacgttccgtctacaactgctccggcgaggcttgccggggacataatcggtcccctttagttcgtaggccttctttacagatgaataccagcatctggtacaaccggagcgacgtgttcgaagcttggcgtttattactgacatccgctccctctttagctaccagccccgcctttcgttatgatttattagatctgactcgtcaagctgtgcaagaactggtgtctttatactacgaggaagctcggagcgcctatttatccaaagagctggcctctttactgagggctggaggcgtgctggcttatgagctgctccccgctttagatgaggttttagctagcgactctcgttttttactgggatcttggctggagcaagctcgtgccgctgccgtgagcgaagccgaggccgatttctatgagcagaactcccggtaccagctgacactctggggccccgagggcaacattctggactacgccaacaagcagctggctggactggtggccaactactacacccctcgttggaggctgtttttagaagctctggtcgactccgtggcccaaggtatccccttccaacagcaccagttcgacaagaatgtgttccagctggaacaagctttcgtgctgtccaaacaaaggtacccctcccagccccggggagacacagtggatctggccaagaagatctttttaaagtattaccctcggtgggtggctggaagctgg

SEQ ID NO: 33 - protein, 720 aa, Artificial Sequence
  amino acid sequence of  hNAGLU mutant type 12
DEAREAAAVRALVARLLGPGPAADFSVSVERALAAKPGLDTYSLGGGGAARVRIRGSTGVAAAAGLHRYLRDFCGCHVAWSGSQLRLPRPLPAVPGELTEATPNRYRYYQNVCTQSYSFVWWDWARWEREIDWMALNGINLALAWSGQEAIWQRVYLALGLTQAEINEFFTGPAFLAWGRMGNLHTWDGPLPPSWHIKQLYLQHRVLDRMRSFGMTPVLPAFAGHVPEAVTRVFPQVNVTKMGSWGHFNCSYSCSFLLAPEDPIFPIIGSLFLRELIKEFGTDHIYGADTFNEMQPPSSEPSYLAAATTAVYEAMTAVDTEAVWLLQGWLFQHQPQFWGPAQIRAVLGAVPRGRLLVLDLFAESQPVYTRTASFQGQPFIWCMLHNFGGNHGLFGALEAVNGGPEAARLFPNSTMVGTGMAPEGISQNEVVYSLMAELGWRKDPVPDLAAWVTSFAARRYGVSHPDAGAAWRLLLRSVYNCSGEACRGHNRSPLVRRPSLQMNTSIWYNRSDVFEAWRLLLTSAPSLATSPAFRYDLLDLTRQAVQELVSLYYEEARSAYLSKELASLLRAGGVLAYELLPALDEVLASDSRFLLGSWLEQARAAAVSEAEADFYEQNSKYQLTLWGPEGNILDYANKQLAGLVANYYTPRWRLFLEALVDSVAQGIPFQQHQFDKNVFQLEQAFVLSKQRYPSQPRGDTVDLAKKIFLKYYPRWVAGSW

SEQ ID NO: 34 - DNA, 2229 bp, Artificial Sequence
  nucleic acid sequence coding hNAGLU mutant type 12, synthetic sequence
atggaggctgtggccgtcgccgccgctgtgggcgtgctgctgctggctggcgctggcggcgccgccggcgacgaggctagggaagccgccgccgtgcgggccctcgtggctaggctgctgggccccggtcccgctgccgatttttccgtgagcgtcgagagggccctcgctgctaagcccggtttagacacctactccctcggcggaggaggagctgctagggttcgtattcgtggatccactggtgtggccgctgctgctggactccatcgttatttacgggatttctgtggatgccacgtggcttggagcggcagccaactgaggctccctaggcctctgcccgctgtccccggtgaactgaccgaggctacccccaatcggtaccggtactaccagaacgtgtgcacccaaagctattccttcgtgtggtgggactgggctcgttgggaaagggagatcgactggatggccctcaacggaattaatctggctttagcttggtccggccaagaggccatttggcagagggtgtacctcgctttaggtttaacacaagctgagatcaacgaattcttcaccggccccgcttttctcgcttggggacggatgggcaatttacacacttgggatggccctctccccccttcttggcacattaagcaactgtatttacagcatcgtgtgctcgatcggatgaggtccttcggcatgacacccgtgctccccgcttttgctggccacgtccccgaagctgtcactcgtgtgtttcctcaagttaacgtgacaaagatgggctcttggggccactttaactgcagctacagctgttcctttttactggcccccgaggatcccatttttcccatcatcggctccctctttttaagggagctgatcaaagagttcggcaccgaccacatttacggcgccgacacctttaacgagatgcagccccctagcagcgagcctagctatttagctgctgccaccacagccgtctatgaggccatgaccgccgtggacaccgaagctgtgtggctgctgcaaggttggctgttccagcaccagcctcagttctggggccccgctcaaattcgtgccgtgctgggcgccgtgcctcggggtcgtctgctggtcctcgatctgttcgctgagtcccaacccgtttacacaaggacagcctccttccaaggtcagcccttcatctggtgcatgctgcacaactttggcggaaaccacggactgttcggagctttagaggctgtgaatggcggacccgaagctgcccggctgttccccaactccaccatggtgggaaccggaatggcccccgaaggcatttcccagaatgaggtggtctacagcctcatggccgagctcggatggcggaaggatcccgttcccgatttagctgcttgggtgacctccttcgctgctcggaggtatggcgtgtcccatcccgatgccggagctgcttggaggttattattacgttccgtctacaactgctccggcgaggcttgccggggacataatcggtcccctttagttcgtaggccttctttacagatgaataccagcatctggtacaaccggagcgacgtgttcgaagcttggcgtttattactgacatccgctccctctttagctaccagccccgcctttcgttatgatttattagatctgactcgtcaagctgtgcaagaactggtgtctttatactacgaggaagctcggagcgcctatttatccaaagagctggcctctttactgagggctggaggcgtgctggcttatgagctgctccccgctttagatgaggttttagctagcgactctcgttttttactgggatcttggctggagcaagctcgtgccgctgccgtgagcgaagccgaggccgatttctatgagcagaactccaagtaccagctgacactctggggccccgagggcaacattctggactacgccaacaagcagctggctggactggtggccaactactacacccctcgttggaggctgtttttagaagctctggtcgactccgtggcccaaggtatccccttccaacagcaccagttcgacaagaatgtgttccagctggaacaagctttcgtgctgtccaaacaaaggtacccctcccagccccggggagacacagtggatctggccaagaagatctttttaaagtattaccctcggtgggtggctggaagctgg

SEQ ID NO: 35 - protein, 721 aa, Artificial Sequence
  amino acid sequence of  hNAGLU mutant type 13
DEAREAAAVRALVARLLGPGPAADFSVSVERALAAKPGLDTYSLSGGGGAARVRIRGSTGVAAAAGLHRYLRDFCGCHVAWSGSQLRLPRPLPAVPGELTEATPNRYRYYQNVCTQSYSFVWWDWARWEREIDWMALNGINLALAWSGQEAIWQRVYLALGLTQAEINEFFTGPAFLAWGRMGNLHTWDGPLPPSWHIKQLYLQHRVLDRMRSFGMTPVLPAFAGHVPEAVTRVFPQVNVTKMGSWGHFNCSYSCSFLLAPEDPIFPIIGSLFLRELIKEFGTDHIYGADTFNEMQPPSSEPSYLAAATTAVYEAMTAVDTEAVWLLQGWLFQHQPQFWGPAQIRAVLGAVPRGRLLVLDLFAESQPVYTRTASFQGQPFIWCMLHNFGGNHGLFGALEAVNGGPEAARLFPNSTMVGTGMAPEGISQNEVVYSLMAELGWRKDPVPDLAAWVTSFAARRYGVSHPDAGAAWRLLLRSVYNCSGEACRGHNRSPLVRRPSLQMNTSIWYNRSDVFEAWRLLLTSAPSLATSPAFRYDLLDLTRQAVQELVSLYYEEARSAYLSKELASLLRAGGVLAYELLPALDEVLASDSRFLLGSWLEQARAAAVSEAEADFYEQNSRYQLTLWGPEGNILDYANKQLAGLVANYYTPRWRLFLEALVDSVAQGIPFQQHQFDKNVFQLEQAFVLSKQRYPSQPRGDTVDLAKKIFLKYYPRWVAGSW

SEQ ID NO: 36 - DNA, 2232 bp, Artificial Sequence
  nucleic acid sequence coding hNAGLU mutant type 13, synthetic sequence
atggaggctgtggccgtcgccgccgctgtgggcgtgctgctgctggctggcgctggcggcgccgccggcgacgaggctagggaagccgccgccgtgcgggccctcgtggctaggctgctgggccccggtcccgctgccgatttttccgtgagcgtcgagagggccctcgctgctaagcccggtttagacacctactccctctctggcggaggaggagctgctagggttcgtattcgtggatccactggtgtggccgctgctgctggactccatcgttatttacgggatttctgtggatgccacgtggcttggagcggcagccaactgaggctccctaggcctctgcccgctgtccccggtgaactgaccgaggctacccccaatcggtaccggtactaccagaacgtgtgcacccaaagctattccttcgtgtggtgggactgggctcgttgggaaagggagatcgactggatggccctcaacggaattaatctggctttagcttggtccggccaagaggccatttggcagagggtgtacctcgctttaggtttaacacaagctgagatcaacgaattcttcaccggccccgcttttctcgcttggggacggatgggcaatttacacacttgggatggccctctccccccttcttggcacattaagcaactgtatttacagcatcgtgtgctcgatcggatgaggtccttcggcatgacacccgtgctccccgcttttgctggccacgtccccgaagctgtcactcgtgtgtttcctcaagttaacgtgacaaagatgggctcttggggccactttaactgcagctacagctgttcctttttactggcccccgaggatcccatttttcccatcatcggctccctctttttaagggagctgatcaaagagttcggcaccgaccacatttacggcgccgacacctttaacgagatgcagccccctagcagcgagcctagctatttagctgctgccaccacagccgtctatgaggccatgaccgccgtggacaccgaagctgtgtggctgctgcaaggttggctgttccagcaccagcctcagttctggggccccgctcaaattcgtgccgtgctgggcgccgtgcctcggggtcgtctgctggtcctcgatctgttcgctgagtcccaacccgtttacacaaggacagcctccttccaaggtcagcccttcatctggtgcatgctgcacaactttggcggaaaccacggactgttcggagctttagaggctgtgaatggcggacccgaagctgcccggctgttccccaactccaccatggtgggaaccggaatggcccccgaaggcatttcccagaatgaggtggtctacagcctcatggccgagctcggatggcggaaggatcccgttcccgatttagctgcttgggtgacctccttcgctgctcggaggtatggcgtgtcccatcccgatgccggagctgcttggaggttattattacgttccgtctacaactgctccggcgaggcttgccggggacataatcggtcccctttagttcgtaggccttctttacagatgaataccagcatctggtacaaccggagcgacgtgttcgaagcttggcgtttattactgacatccgctccctctttagctaccagccccgcctttcgttatgatttattagatctgactcgtcaagctgtgcaagaactggtgtctttatactacgaggaagctcggagcgcctatttatccaaagagctggcctctttactgagggctggaggcgtgctggcttatgagctgctccccgctttagatgaggttttagctagcgactctcgttttttactgggatcttggctggagcaagctcgtgccgctgccgtgagcgaagccgaggccgatttctatgagcagaactcccggtaccagctgacactctggggccccgagggcaacattctggactacgccaacaagcagctggctggactggtggccaactactacacccctcgttggaggctgtttttagaagctctggtcgactccgtggcccaaggtatccccttccaacagcaccagttcgacaagaatgtgttccagctggaacaagctttcgtgctgtccaaacaaaggtacccctcccagccccggggagacacagtggatctggccaagaagatctttttaaagtattaccctcggtgggtggctggaagctgg

SEQ ID NO: 37 - protein, 721 aa, Artificial Sequence
  amino acid sequence of  hNAGLU mutant type 14
DEAREAAAVRALVARLLGPGPAADFSVSVERALAAKPGLDTYSLSGGGGAARVRVRGSTGVAAAAGLHRYLRDFCGCHVAWSGSQLRLPRPLPAVPGELTEATPNRYRYYQNVCTQSYSFVWWDWARWEREIDWMALNGINLALAWSGQEAIWQRVYLALGLTQAEINEFFTGPAFLAWGRMGNLHTWDGPLPPSWHIKQLYLQHRVLDRMRSFGMTPVLPAFAGHVPEAVTRVFPQVNVTKMGSWGHFNCSYSCSFLLAPEDPIFPIIGSLFLRELIKEFGTDHIYGADTFNEMQPPSSEPSYLAAATTAVYEAMTAVDTEAVWLLQGWLFQHQPQFWGPAQIRAVLGAVPRGRLLVLDLFAESQPVYTRTASFQGQPFIWCMLHNFGGNHGLFGALEAVNGGPEAARLFPNSTMVGTGMAPEGISQNEVVYSLMAELGWRKDPVPDLAAWVTSFAARRYGVSHPDAGAAWRLLLRSVYNCSGEACRGHNRSPLVRRPSLQMNTSIWYNRSDVFEAWRLLLTSAPSLATSPAFRYDLLDLTRQAVQELVSLYYEEARSAYLSKELASLLRAGGVLAYELLPALDEVLASDSRFLLGSWLEQARAAAVSEAEADFYEQNSKYQLTLWGPEGNILDYANKQLAGLVANYYTPRWRLFLEALVDSVAQGIPFQQHQFDKNVFQLEQAFVLSKQRYPSQPRGDTVDLAKKIFLKYYPRWVAGSW

SEQ ID NO: 38 - DNA, 2232 bp, Artificial Sequence
  nucleic acid sequence coding hNAGLU mutant type 14, synthetic sequence
atggaggctgtggccgtcgccgccgctgtgggcgtgctgctgctggctggcgctggcggcgccgccggcgacgaggctagggaagccgccgccgtgcgggccctcgtggctaggctgctgggccccggtcccgctgccgatttttccgtgagcgtcgagagggccctcgctgctaagcccggtttagacacctactccctctctggcggaggaggagctgctagggttcgtgttcgtggatccactggtgtggccgctgctgctggactccatcgttatttacgggatttctgtggatgccacgtggcttggagcggcagccaactgaggctccctaggcctctgcccgctgtccccggtgaactgaccgaggctacccccaatcggtaccggtactaccagaacgtgtgcacccaaagctattccttcgtgtggtgggactgggctcgttgggaaagggagatcgactggatggccctcaacggaattaatctggctttagcttggtccggccaagaggccatttggcagagggtgtacctcgctttaggtttaacacaagctgagatcaacgaattcttcaccggccccgcttttctcgcttggggacggatgggcaatttacacacttgggatggccctctccccccttcttggcacattaagcaactgtatttacagcatcgtgtgctcgatcggatgaggtccttcggcatgacacccgtgctccccgcttttgctggccacgtccccgaagctgtcactcgtgtgtttcctcaagttaacgtgacaaagatgggctcttggggccactttaactgcagctacagctgttcctttttactggcccccgaggatcccatttttcccatcatcggctccctctttttaagggagctgatcaaagagttcggcaccgaccacatttacggcgccgacacctttaacgagatgcagccccctagcagcgagcctagctatttagctgctgccaccacagccgtctatgaggccatgaccgccgtggacaccgaagctgtgtggctgctgcaaggttggctgttccagcaccagcctcagttctggggccccgctcaaattcgtgccgtgctgggcgccgtgcctcggggtcgtctgctggtcctcgatctgttcgctgagtcccaacccgtttacacaaggacagcctccttccaaggtcagcccttcatctggtgcatgctgcacaactttggcggaaaccacggactgttcggagctttagaggctgtgaatggcggacccgaagctgcccggctgttccccaactccaccatggtgggaaccggaatggcccccgaaggcatttcccagaatgaggtggtctacagcctcatggccgagctcggatggcggaaggatcccgttcccgatttagctgcttgggtgacctccttcgctgctcggaggtatggcgtgtcccatcccgatgccggagctgcttggaggttattattacgttccgtctacaactgctccggcgaggcttgccggggacataatcggtcccctttagttcgtaggccttctttacagatgaataccagcatctggtacaaccggagcgacgtgttcgaagcttggcgtttattactgacatccgctccctctttagctaccagccccgcctttcgttatgatttattagatctgactcgtcaagctgtgcaagaactggtgtctttatactacgaggaagctcggagcgcctatttatccaaagagctggcctctttactgagggctggaggcgtgctggcttatgagctgctccccgctttagatgaggttttagctagcgactctcgttttttactgggatcttggctggagcaagctcgtgccgctgccgtgagcgaagccgaggccgatttctatgagcagaactccaagtaccagctgacactctggggccccgagggcaacattctggactacgccaacaagcagctggctggactggtggccaactactacacccctcgttggaggctgtttttagaagctctggtcgactccgtggcccaaggtatccccttccaacagcaccagttcgacaagaatgtgttccagctggaacaagctttcgtgctgtccaaacaaaggtacccctcccagccccggggagacacagtggatctggccaagaagatctttttaaagtattaccctcggtgggtggctggaagctgg

SEQ ID NO: 39 - protein, 721 aa, Artificial Sequence
  amino acid sequence of  hNAGLU mutant type 15
DEAREAAAVRALVARLLGPGPAADFSVSVERALAAKPGLDTYSLSGGGGAARVRIRGSTGVAAAAGLHRYLRDFCGCHVAWSGSQLRLPRPLPAVPGELTEATPNRYRYYQNVCTQSYSFVWWDWARWEREIDWMALNGINLALAWSGQEAIWQRVYLALGLTQAEINEFFTGPAFLAWGRMGNLHTWDGPLPPSWHIKQLYLQHRVLDRMRSFGMTPVLPAFAGHVPEAVTRVFPQVNVTKMGSWGHFNCSYSCSFLLAPEDPIFPIIGSLFLRELIKEFGTDHIYGADTFNEMQPPSSEPSYLAAATTAVYEAMTAVDTEAVWLLQGWLFQHQPQFWGPAQIRAVLGAVPRGRLLVLDLFAESQPVYTRTASFQGQPFIWCMLHNFGGNHGLFGALEAVNGGPEAARLFPNSTMVGTGMAPEGISQNEVVYSLMAELGWRKDPVPDLAAWVTSFAARRYGVSHPDAGAAWRLLLRSVYNCSGEACRGHNRSPLVRRPSLQMNTSIWYNRSDVFEAWRLLLTSAPSLATSPAFRYDLLDLTRQAVQELVSLYYEEARSAYLSKELASLLRAGGVLAYELLPALDEVLASDSRFLLGSWLEQARAAAVSEAEADFYEQNSKYQLTLWGPEGNILDYANKQLAGLVANYYTPRWRLFLEALVDSVAQGIPFQQHQFDKNVFQLEQAFVLSKQRYPSQPRGDTVDLAKKIFLKYYPRWVAGSW

SEQ ID NO: 40 - DNA, 2232 bp, Artificial Sequence
  nucleic acid sequence coding hNAGLU mutant type 15, synthetic sequence
atggaggctgtggccgtcgccgccgctgtgggcgtgctgctgctggctggcgctggcggcgccgccggcgacgaggctagggaagccgccgccgtgcgggccctcgtggctaggctgctgggccccggtcccgctgccgatttttccgtgagcgtcgagagggccctcgctgctaagcccggtttagacacctactccctctctggcggaggaggagctgctagggttcgtattcgtggatccactggtgtggccgctgctgctggactccatcgttatttacgggatttctgtggatgccacgtggcttggagcggcagccaactgaggctccctaggcctctgcccgctgtccccggtgaactgaccgaggctacccccaatcggtaccggtactaccagaacgtgtgcacccaaagctattccttcgtgtggtgggactgggctcgttgggaaagggagatcgactggatggccctcaacggaattaatctggctttagcttggtccggccaagaggccatttggcagagggtgtacctcgctttaggtttaacacaagctgagatcaacgaattcttcaccggccccgcttttctcgcttggggacggatgggcaatttacacacttgggatggccctctccccccttcttggcacattaagcaactgtatttacagcatcgtgtgctcgatcggatgaggtccttcggcatgacacccgtgctccccgcttttgctggccacgtccccgaagctgtcactcgtgtgtttcctcaagttaacgtgacaaagatgggctcttggggccactttaactgcagctacagctgttcctttttactggcccccgaggatcccatttttcccatcatcggctccctctttttaagggagctgatcaaagagttcggcaccgaccacatttacggcgccgacacctttaacgagatgcagccccctagcagcgagcctagctatttagctgctgccaccacagccgtctatgaggccatgaccgccgtggacaccgaagctgtgtggctgctgcaaggttggctgttccagcaccagcctcagttctggggccccgctcaaattcgtgccgtgctgggcgccgtgcctcggggtcgtctgctggtcctcgatctgttcgctgagtcccaacccgtttacacaaggacagcctccttccaaggtcagcccttcatctggtgcatgctgcacaactttggcggaaaccacggactgttcggagctttagaggctgtgaatggcggacccgaagctgcccggctgttccccaactccaccatggtgggaaccggaatggcccccgaaggcatttcccagaatgaggtggtctacagcctcatggccgagctcggatggcggaaggatcccgttcccgatttagctgcttgggtgacctccttcgctgctcggaggtatggcgtgtcccatcccgatgccggagctgcttggaggttattattacgttccgtctacaactgctccggcgaggcttgccggggacataatcggtcccctttagttcgtaggccttctttacagatgaataccagcatctggtacaaccggagcgacgtgttcgaagcttggcgtttattactgacatccgctccctctttagctaccagccccgcctttcgttatgatttattagatctgactcgtcaagctgtgcaagaactggtgtctttatactacgaggaagctcggagcgcctatttatccaaagagctggcctctttactgagggctggaggcgtgctggcttatgagctgctccccgctttagatgaggttttagctagcgactctcgttttttactgggatcttggctggagcaagctcgtgccgctgccgtgagcgaagccgaggccgatttctatgagcagaactccaagtaccagctgacactctggggccccgagggcaacattctggactacgccaacaagcagctggctggactggtggccaactactacacccctcgttggaggctgtttttagaagctctggtcgactccgtggcccaaggtatccccttccaacagcaccagttcgacaagaatgtgttccagctggaacaagctttcgtgctgtccaaacaaaggtacccctcccagccccggggagacacagtggatctggccaagaagatctttttaaagtattaccctcggtgggtggctggaagctgg

SEQ ID NO: 41 - DNA, 2285 bp, Artificial Sequence
  nucleic acid sequence containing a gene coding hNAGLU, synthetic sequence
ttttacgcgtcgccaccatggaggctgtggccgtcgccgccgctgtgggcgtgctgctgctggctggcgctggcggcgccgccggcgacgaggctagggaagccgccgccgtgcgggccctcgtggctaggctgctgggccccggtcccgctgccgatttttccgtgagcgtcgagagggccctcgctgctaagcccggtttagacacctactccctcggcggaggaggagctgctagggttcgtgttcgtggatccactggtgtggccgctgctgctggactccatcgttatttacgggatttctgtggatgccacgtggcttggagcggcagccaactgaggctccctaggcctctgcccgctgtccccggtgaactgaccgaggctacccccaatcggtaccggtactaccagaacgtgtgcacccaaagctattccttcgtgtggtgggactgggctcgttgggaaagggagatcgactggatggccctcaacggaattaatctggctttagcttggtccggccaagaggccatttggcagagggtgtacctcgctttaggtttaacacaagctgagatcaacgaattcttcaccggccccgcttttctcgcttggggacggatgggcaatttacacacttgggatggccctctccccccttcttggcacattaagcaactgtatttacagcatcgtgtgctcgatcagatgaggtccttcggcatgacacccgtgctccccgcttttgctggccacgtccccgaagctgtcactcgtgtgtttcctcaagttaacgtgacaaagatgggctcttggggccactttaactgcagctacagctgttcctttttactggcccccgaggatcccatttttcccatcatcggctccctctttttaagggagctgatcaaagagttcggcaccgaccacatttacggcgccgacacctttaacgagatgcagccccctagcagcgagcctagctatttagctgctgccaccacagccgtctatgaggccatgaccgccgtggacaccgaagctgtgtggctgctgcaaggttggctgttccagcaccagcctcagttctggggccccgctcaaattcgtgccgtgctgggcgccgtgcctcggggtcgtctgctggtcctcgatctgttcgctgagtcccaacccgtttacacaaggacagcctccttccaaggtcagcccttcatctggtgcatgctgcacaactttggcggaaaccacggactgttcggagctttagaggctgtgaatggcggacccgaagctgcccggctgttccccaactccaccatggtgggaaccggaatggcccccgaaggcatttcccagaatgaggtggtctacagcctcatggccgagctcggatggcggaaggatcccgttcccgatttagctgcttgggtgacctccttcgctgctcggaggtatggcgtgtcccatcccgatgccggagctgcttggaggttattattacgttccgtctacaactgctccggcgaggcttgccggggacataatcggtcccctttagttcgtaggccttctttacagatgaataccagcatctggtacaaccggagcgacgtgttcgaagcttggcgtttattactgacatccgctccctctttagctaccagccccgcctttcgttatgatttattagatctgactcgtcaagctgtgcaagaactggtgtctttatactacgaggaagctcggagcgcctatttatccaaagagctggcctctttactgagggctggaggcgtgctggcttatgagctgctccccgctttagatgaggttttagctagcgactctcgttttttactgggatcttggctggagcaagctcgtgccgctgccgtgagcgaagccgaggccgatttctatgagcagaactcccggtaccagctgacactctggggccccgagggcaacattctggactacgccaacaagcagctggctggactggtggccaactactacacccctcgttggaggctgtttttagaagctctggtcgactccgtggcccaaggtatccccttccaacagcaccagttcgacaagaatgtgttccagctggaacaagctttcgtgctgtccaaacaaaggtacccctcccagccccggggagacacagtggatctggccaagaagatctttttaaagtattaccctcggtgggtggctggaagctggcatcaccatcaccatcactaagcggccgcaaagacagaa

SEQ ID NO: 42 - DNA, 24 bp, Artificial Sequence
  MluI addition 5' primer
ttttacgcgtcgccaccatggagg

SEQ ID NO: 43 - DNA, 58 bp, Artificial Sequence
  His Tag-NotI addition 5' primer
ttctgtctttgcggccgcttagtgatggtgatggtgatgccagcttccagccacccac

SEQ ID NO: 44 - DNA, 27 bp, Artificial Sequence
  3' primer for introducing K59E/P60S mutation, synthetic sequence
gtgtctaaaccggactcagcagcgagg

SEQ ID NO: 45 - DNA, 23 bp, Artificial Sequence
  3' primer for introducing L67_G68insS mutation, synthetic sequence
ctcctccgccagagagggagtag

SEQ ID NO: 46 - DNA, 25 bp, Artificial Sequence
  3' primer for introducing R152Q mutation, synthetic sequence
cagtcgatctcctgttcccaacgag

SEQ ID NO: 47 - DNA, 26 bp, Artificial Sequence
  3' primer for introducing Q232R mutation, synthetic sequence
gaaggacctcatccgatcgagcacac

SEQ ID NO: 48 - DNA, 22 bp, Artificial Sequence
  3' primer for introducing E251K mutation, synthetic sequence
gagtgacagctttggggacgtg

SEQ ID NO: 49 - DNA, 26 bp, Artificial Sequence
  3' primer for introducing T263V mutation, synthetic sequence
gagcccatcttgaccacgttaacttg

SEQ ID NO: 50 - DNA, 25 bp, Artificial Sequence
  3' primer for introducing T343P/E344D mutation, synthetic sequence
gccacacagcgtcggggtccacggc

SEQ ID NO: 51 - DNA, 29 bp, Artificial Sequence
  5' primer for introducing S528A/I529V mutation, synthetic sequence
cagatgaataccgccgtctggtacaaccg

SEQ ID NO: 52 - DNA, 29 bp, Artificial Sequence
  5' primer for introducing S549N/A551T mutation, synthetic sequence
catccgctcccaatttaactaccagcccc

SEQ ID NO: 53 - DNA, 24 bp, Artificial Sequence
  5' primer for introducing D636Q mutation, synthetic sequence
gccgaggcccagttctatgagcag

SEQ ID NO: 54 - DNA, 25 bp, Artificial Sequence
  3' primer for introducing H227K mutation, synthetic sequence
cgagcacacgcttctgtaaatacag

SEQ ID NO: 55 - DNA, 23 bp, Artificial Sequence
  3' primer for introducing V77I mutation, synthetic sequence
ggatccacgaatacgaaccctag

SEQ ID NO: 56 - DNA, 22 bp, Artificial Sequence
  5' primer for introducing R643K mutation, synthetic sequence
gcagaactccaagtaccagctg

SEQ ID NO: 57 - protein, 760 aa, Homo sapiens
MMDQARSAFSNLFGGEPLSYTRFSLARQVDGDNSHVEMKLAVDEEENADNNTKANVTKPKRCSGSICYGTIAVIVFFLIGFMIGYLGYCKGVEPKTECERLAGTESPVREEPGEDFPAARRLYWDDLKRKLSEKLDSTDFTGTIKLLNENSYVPREAGSQKDENLALYVENQFREFKLSKVWRDQHFVKIQVKDSAQNSVIIVDKNGRLVYLVENPGGYVAYSKAATVTGKLVHANFGTKKDFEDLYTPVNGSIVIVRAGKITFAEKVANAESLNAIGVLIYMDQTKFPIVNAELSFFGHAHLGTGDPYTPGFPSFNHTQFPPSRSSGLPNIPVQTISRAAAEKLFGNMEGDCPSDWKTDSTCRMVTSESKNVKLTVSNVLKEIKILNIFGVIKGFVEPDHYVVVGAQRDAWGPGAAKSGVGTALLLKLAQMFSDMVLKDGFQPSRSIIFASWSAGDFGSVGATEWLEGYLSSLHLKAFTYINLDKAVLGTSNFKVSASPLLYTLIEKTMQNVKHPVTGQFLYQDSNWASKVEKLTLDNAAFPFLAYSGIPAVSFCFCEDTDYPYLGTTMDTYKELIERIPELNKVARAAAEVAGQFVIKLTHDVELNLDYERYNSQLLSFVRDLNQYRADIKEMGLSLQWLYSARGDFFRATSRLTTDFGNAEKTDRFVMKKLNDRVMRVEYHFLSPYVSPKESPFRHVFWGSGSHTLPALLENLKLRKQNNGAFNETLFRNQLALATWTIQGAANALSGDVWDIDNEF

SEQ ID NO: 58 - protein, 5 aa, Artificial Sequence
  amino acid sequence of an exemplified linker 1
GGGGS

SEQ ID NO: 59 - protein, 6 aa, Artificial Sequence
  amino acid sequence of an exemplified linker 2
GGGGGS

SEQ ID NO: 60 - protein, 5 aa, Artificial Sequence
  amino acid sequence of an exemplified linker 3
SGGGG

SEQ ID NO: 61 - protein, 219 aa, Artificial Sequence
  amino acid sequence of the light-chain of anti-hTfR antibody
DIVMTQTPLSLSVTPGQPASISCRSSQSLVHSNGNTYLHWYLQKPGQSPQLLIYKVSNRFSGVPDRFSGSGSGTDFTLKISRVEAEDVGVYYCSQSTHVPWTFGQGTKVEIKRTVAAPSVFIFPPSDEQLKSGTASVVCLLNNFYPREAKVQWKVDNALQSGNSQESVTEQDSKDSTYSLSSTLTLSKADYEKHKVYACEVTHQGLSSPVTKSFNRGEC

SEQ ID NO: 62 - protein, 448 aa, Artificial Sequence
  amino acid sequence of the heavy-chain of anti-hTfR antibody
EVQLVQSGAEVKKPGESLKISCKGSGYSFTNYWLGWVRQMPGKGLEWMGDIYPGGDYPTYSEKFKVQVTISADKSISTAYLQWSSLKASDTAMYYCARSGNYDEVAYWGQGTLVTVSSASTKGPSVFPLAPSSKSTSGGTAALGCLVKDYFPEPVTVSWNSGALTSGVHTFPAVLQSSGLYSLSSVVTVPSSSLGTQTYICNVNHKPSNTKVDKKVEPKSCDKTHTCPPCPAPELLGGPSVFLFPPKPKDTLMISRTPEVTCVVVDVSHEDPEVKFNWYVDGVEVHNAKTKPREEQYNSTYRVVSVLTVLHQDWLNGKEYKCKVSNKALPAPIEKTISKAKGQPREPQVYTLPPSRDELTKNQVSLTCLVKGFYPSDIAVEWESNGQPENNYKTTPPVLDSDGSFFLYSKLTVDKSRWQQGNVFSCSVMHEALHNHYTQKSLSLSPGK

SEQ ID NO: 63 - protein, 226 aa, Artificial Sequence
  amino acid sequence of Fab heavy chain of anti-hTfR antibody
EVQLVQSGAEVKKPGESLKISCKGSGYSFMNYWLGWVRQMPGKGLEWMGDIYPGGDYPTYSEKFKVQVTISADKSISTAYLQLSSLKASDTAMYYCARSGNYDEVAYWGQGTLVTVSSASTKGPSVFPLAPSSKSTSGGTAALGCLVKDYFPEPVTVSWNSGALTSGVHTFPAVLQSSGLYSLSSVVTVPSSSLGTQTYICNVNHKPSNTKVDKKVEPKSCDKTHT

SEQ ID NO: 64 - protein, 962 aa, Artificial Sequence
  amino acid sequence of fusion protein of hNAGLU mutant type 9 and Fab heavy chain of anti-hTfR antibody (1)
EVQLVQSGAEVKKPGESLKISCKGSGYSFMNYWLGWVRQMPGKGLEWMGDIYPGGDYPTYSEKFKVQVTISADKSISTAYLQLSSLKASDTAMYYCARSGNYDEVAYWGQGTLVTVSSASTKGPSVFPLAPSSKSTSGGTAALGCLVKDYFPEPVTVSWNSGALTSGVHTFPAVLQSSGLYSLSSVVTVPSSSLGTQTYICNVNHKPSNTKVDKKVEPKSCDKTHTGGGGSGGGGSGGGGSDEAREAAAVRALVARLLGPGPAADFSVSVERALAAKPGLDTYSLSGGGGAARVRVRGSTGVAAAAGLHRYLRDFCGCHVAWSGSQLRLPRPLPAVPGELTEATPNRYRYYQNVCTQSYSFVWWDWARWEREIDWMALNGINLALAWSGQEAIWQRVYLALGLTQAEINEFFTGPAFLAWGRMGNLHTWDGPLPPSWHIKQLYLQHRVLDRMRSFGMTPVLPAFAGHVPEAVTRVFPQVNVTKMGSWGHFNCSYSCSFLLAPEDPIFPIIGSLFLRELIKEFGTDHIYGADTFNEMQPPSSEPSYLAAATTAVYEAMTAVDTEAVWLLQGWLFQHQPQFWGPAQIRAVLGAVPRGRLLVLDLFAESQPVYTRTASFQGQPFIWCMLHNFGGNHGLFGALEAVNGGPEAARLFPNSTMVGTGMAPEGISQNEVVYSLMAELGWRKDPVPDLAAWVTSFAARRYGVSHPDAGAAWRLLLRSVYNCSGEACRGHNRSPLVRRPSLQMNTSIWYNRSDVFEAWRLLLTSAPSLATSPAFRYDLLDLTRQAVQELVSLYYEEARSAYLSKELASLLRAGGVLAYELLPALDEVLASDSRFLLGSWLEQARAAAVSEAEADFYEQNSRYQLTLWGPEGNILDYANKQLAGLVANYYTPRWRLFLEALVDSVAQGIPFQQHQFDKNVFQLEQAFVLSKQRYPSQPRGDTVDLAKKIFLKYYPRWVAGSW

SEQ ID NO: 65 - protein, 962 aa, Artificial Sequence
  amino acid sequence of fusion protein of hNAGLU mutant type 9 and Fab heavy chain of anti-hTfR antibody (2)
DEAREAAAVRALVARLLGPGPAADFSVSVERALAAKPGLDTYSLSGGGGAARVRVRGSTGVAAAAGLHRYLRDFCGCHVAWSGSQLRLPRPLPAVPGELTEATPNRYRYYQNVCTQSYSFVWWDWARWEREIDWMALNGINLALAWSGQEAIWQRVYLALGLTQAEINEFFTGPAFLAWGRMGNLHTWDGPLPPSWHIKQLYLQHRVLDRMRSFGMTPVLPAFAGHVPEAVTRVFPQVNVTKMGSWGHFNCSYSCSFLLAPEDPIFPIIGSLFLRELIKEFGTDHIYGADTFNEMQPPSSEPSYLAAATTAVYEAMTAVDTEAVWLLQGWLFQHQPQFWGPAQIRAVLGAVPRGRLLVLDLFAESQPVYTRTASFQGQPFIWCMLHNFGGNHGLFGALEAVNGGPEAARLFPNSTMVGTGMAPEGISQNEVVYSLMAELGWRKDPVPDLAAWVTSFAARRYGVSHPDAGAAWRLLLRSVYNCSGEACRGHNRSPLVRRPSLQMNTSIWYNRSDVFEAWRLLLTSAPSLATSPAFRYDLLDLTRQAVQELVSLYYEEARSAYLSKELASLLRAGGVLAYELLPALDEVLASDSRFLLGSWLEQARAAAVSEAEADFYEQNSRYQLTLWGPEGNILDYANKQLAGLVANYYTPRWRLFLEALVDSVAQGIPFQQHQFDKNVFQLEQAFVLSKQRYPSQPRGDTVDLAKKIFLKYYPRWVAGSWGGGGSGGGGSGGGGSEVQLVQSGAEVKKPGESLKISCKGSGYSFMNYWLGWVRQMPGKGLEWMGDIYPGGDYPTYSEKFKVQVTISADKSISTAYLQLSSLKASDTAMYYCARSGNYDEVAYWGQGTLVTVSSASTKGPSVFPLAPSSKSTSGGTAALGCLVKDYFPEPVTVSWNSGALTSGVHTFPAVLQSSGLYSLSSVVTVPSSSLGTQTYICNVNHKPSNTKVDKKVEPKSCDKTHT

SEQ ID NO: 66 - DNA, 740 bp, Artificial Sequence
  nucleotide sequence encoding the amino acid sequence of the light chain of anti-hTfR antibody, synthetic sequence
acgcgtgccgccaccatgggctggagctggattctgctgttcctcctgagcgtgacagcaggagtgcacagcgacatcgtgatgacccagactcccctgagcctgagcgtgacacctggccagcctgccagcatcagctgcagaagctctcagagcctggtgcacagcaacggcaacacctacctgcactggtatctgcagaagcccggccagagccctcagctgctgatctacaaggtgtccaacagattcagcggcgtgcccgacagattctccggcagcggctctggcaccgacttcaccctgaagatttccagagtggaagccgaggacgtgggcgtgtactactgcagccagagcacccacgtgccctggacattcggccagggcaccaaggtggaaatcaagagaaccgtggccgctcccagcgtgttcatcttcccacctagcgacgagcagctgaagtccggcacagcctctgtcgtgtgcctgctgaacaacttctacccccgcgaggccaaggtgcagtggaaggtggacaacgccctgcagagcggcaacagccaggaaagcgtgaccgagcaggactccaaggacagcacctacagcctgagcagcaccctgaccctgagcaaggccgactacgagaagcacaaggtgtacgcctgcgaagtgacccaccagggcctgtctagccccgtgaccaagagcttcaacagaggcgagtgctaagcggccgc

SEQ ID NO: 67 - protein, 23 aa, Homo sapiens
MEAVAVAAAVGVLLLAGAGGAAG